European Patent Specification EP 2 515 630 B1, published June 5, 2024. Title: GENETIC MARKERS ASSOCIATED WITH DROUGHT TOLERANCE IN MAIZE. Applicant: Syngenta Participations AG Kishore, Venkata K. Altendorf, Paul Prest, Thomas J. Zinselmeier, Chris Wang, Daolong Briggs, Bill Ghandi, Sonali Foster, David Chaulk-Grace, Christine Clarke V, Joseph D. Sessions, Allen Kust, Kari D. Tucker, Jon A. Guitierrez Rojas, Libardo Andres Li, Meijuan Warner, Todd Martin, Nicolas Miller, Robert L. Arbuckle, John Skalla, Dale W. Application PCTUS1062028. The sequence listing filed with the application follows.

SEQUENCE LISTING (413 sequences)

SEQ ID NO: 1 - DNA, 552 bp, Zea mays
  misc_feature (75)..(508): n is a, c, g, or t
  misc_feature (115)..(115): s is c or g
  misc_feature (270)..(483): r is a or g
  misc_feature (301)..(301): y is c or t
tagggtcctgctacaagagatcgccacattttattgctacggaagtccagttgtgtctgtctgtttggtggtcantggnatatggttcggtttttactgctgtaaaaagggactsgggaannaaaaatgcaaactgacttggattttttgttctgttctgcatgaagatgaaatggtagggtcgtcggaggaggacgaagcatgctcgggaggagacacggaggcgacggagccggggcagcaggagcacagctcccgcctggcggaccrtgagctgaaggagatgctgctgaagaagtayagcgggtgcctgagccggctgcggtccgagttcctgaagaagaggaagaaagggaagctgcccaaggacgcgcggtcggcgctcatggactggtggaacacgcactaccgctggccgtaccctacggtaaccatgcatgcatcctggcaaacacgcagcagcagcatcgctcgctggaatgrcagatctgtgaccagcatnnncngncggtgcaggaggaggacaaggtgaggctggcggcggcgactggg

SEQ ID NO: 2 - DNA, 490 bp, Zea mays
  misc_feature (100)..(100): r is a or g
  misc_feature (264)..(271): the sequence nnnnnnn is either caccaagg or is absent
tagccgtcctgcaaacctcctggataaagtttggaccttatttaggaagagaagcaccctggacgagccgcgtggtatcaattcttgccgctctcctccrctttcatcttcttctcccacctacgtttctggtggaaaaaaagtttcaaagcacgaacagagagatgagccagttagatcttttttcaagggatgccttcgttcaatcactattacagctatcgttacatttgatctgaaaacacaaacatggcatctttgtgnnnnnnnntcaatgcaggataaaaagctggatcgctgacaacagatatttgattgtccgttggaaaatattttttcaatggccacagttttagaaaatattttcccaaaattatgtcattactattactagactagcaaagtagataatggcgagcaaccatcaggaaatcttgccatcagtgcagcagaactgcagacccttatattagcgcaccagcagaatcta

SEQ ID NO: 3 - DNA, 427 bp, Zea mays
  misc_feature (18)..(18): d is a or g or t
  misc_feature (49)..(416): n is a, c, g, or t
  misc_feature (216)..(216): k is g or t
cgagtggtttgaggttgdcacacaagtattgaatattgataaatcacanatacntnnacagggcggacaaaggtgacaccattaaagtgtcaggngtttatcaccttgangagaaacagaaggcctcagctgtggctgagctaacccggaggctctcaacaaatcagaacacactcacagtcggnggactgtncacagttgatccccagacagctktgaaggcaagactcaataacactggaacgcttgccgcgcttcttcagcatgagcttaaacccaagtcgctcttgacnatctctggtgaattcgacacaaangccctggacagatccccaaagtttgggttggcgcttgcactgaagccctgatcagatcatcccatgttgattgatgattggtggtgaatcttgaattcnttttttttttt

SEQ ID NO: 4 - DNA, 1020 bp, Zea mays
  misc_feature (503)..(503): r is a or g
cttaatatgtgagttttctaagttagtaatcttatatatttgggcactgtatgcgactgttgttctgacaacccttaagcttatttgatacctgtaatatctttattgatggttaattgcaaatccctgcttgatgcatctcaacttcaagttgttttgtagctggtttagtgcataaaattagtcaaaatattaatataccggtcaccgtcatttcaccttttctcactgacatttctcaaatggagttttgaaagaaggttttacttcacttatatacgtttgcaacaaacatgagtttctaattcactcagattataaaaaaactcggccggggaggaaatgaccgtcttgctggtattatattaagaagagaccgaaacaatggtcctgccgagaaaatccttgaaccctggcccccatcactaacggaccggtgtcaaccgtcaactctgcaacggcccaaccggagggtggcgcataggacatcgtaacccgagacrgagagcgggtggggcacagcgagggaatttttttaaccaagccgaaaaattcgcccctgaggtgttactcggaagcctttaatcactaggttagaggccctttcgcaactcactcagattattgcatgtacagaaattggtcaatgtaactgactttgctagtgtttttagtttcactgaaaaaaggatctcttgcagtaagctggtagcagcagtatggctaatattaagctgtgcctccagtaagggtttggtgctcagtattttgtttttctaattgagtcaaaagtcttatgtataatcttatattaaatgaaattgatgtcatagttcctcaacagatataatcccatttttaaggacgtttaacgtcttattattgcagttacatccaaattttctgtaacttatccaaccttctcttgcaggaacaacaagggagacaaccttactggagcttactaccacaaggtgagcgaattgacaaacacagctgttggggcagagcttacccact

SEQ ID NO: 5 - DNA, 910 bp, Zea mays
  misc_feature (283)..(440): n is a, c, g, or t
  misc_feature (818)..(821): nnnn is cgcg or is absent
  misc_feature (860)..(872): n is a, c, g, or t
acaactacaaggacctcgaagccgaggctgctgcggcgacggaccaggtgccgccgtccatcgtcaaccccctgctcaggacggggtaccacttccagccccccaagaactggatcaatggtaatgtaaagctactaactaatccaccacccaacgtcgtttgaaggtgatgtgtgtgttaagcatctcctgaaatatataagagagcgaggctagtaatcggcttgttgttcagggttttggtttaccacttgtagcctcaactaataaagctatatatatnngagagcgacgagagagaagagacaaaacattcatgagtatggtcagacagactagctagctagacacggcagagaaattacgagagttaaaaaaaantgcgcttgaagggtgaaccaaaacaaaacaactttagtactatgcgtcaacaaannnnngctgtgttcatgtgtcagctagcactagagtcatagtgcgtggccagtgagctgttgtctagcaaccaacgcgaactgaagtttgagagcgtactcgtgttctcgatctcttgcagcgcaaaggtcttcgtacgtgatcaggaatattgcaccatttactgcttaattaattaagtacgtacgtactgtacgtttggctctacctcatcttctaatcttttcggtgctgtcttgtgctctctcggctctgattgcatcgatcggcggcggcgtgaactttgcaacggcggcagatcccaacggtaataagtcgttttccccaccctttttatttcctctaataatgcatcaatattccaactgggtgcatatgcatgnnnncagcgcccatgtactacaaggggtggtaccatttcttcntaccaatacaantcccaagggcgccgtatggggcaacatcgtgtgggcgc

SEQ ID NO: 6 - DNA, 346 bp, Zea mays
  misc_feature (98)..(99): n is a, c, g, or t
  misc_feature (254)..(254): r is a or g
gggcaggcgtgtacaagccgccatacggaggattcgtggacgtcgacgttgaggagcacgagaccatcaatttgagaaccctggtgagtttttttttnnctttttacttttttgctgctttgtccttcagcgatctgctcagttcgtttgtaatttgcacagattgatcactcggtggtggagagcttcggagctgacgggcggatgtgcatcacggctcgagtgtaccctgagcacgcggagacgagcaacarccacatgttcgtgttcaacaatggcacaggcacggtggaggtgtccaagctcgaggcatgggagctcgcggcggcgaccgtaaattccgttg

SEQ ID NO: 7 - DNA, 7437 bp, Zea mays
  misc_feature (4454)..(4474): n is a, c, g, or t
  misc_feature (4497)..(4498): nn is ga or both nucleotides are absent
  misc_feature (4505)..(4969): k is g or t
  misc_feature (4505)..(4969): m is a or c
  misc_feature (4505)..(4969): w is a or t
  misc_feature (4505)..(4969): y is c or t
  misc_feature (4536)..(5309): n is a, c, g, or t
  misc_feature (4979)..(4981): wcy is either act or tcc
aatgtcaagtatatccatttaaatatcattaggtcccgtttgtttcctttcattttaaggaattggaatcttactaataaaataagctatttttttagaatacgagattccaccactttccaaagttatcagataagcctatctcaaattcatggggtgagagatggaaattgattctatagatttacatgttattttcccgatgtacaacttatatcatactctcctaattgcttcgctataacataaatgcactatataactatctctcttatatgatttaggataatatacaaatatattacatatataaatatattaacttaattagttttgtctaaattataattattaaaatggaattcaattccaacgaaacaaacgggcccttacaaaatttctagtatcatttaaccatctattcaacacaccaaagataattggataaaatagcaacactaggacaaatactacatagcacattacatgttccattatatggtcattaaattgtcgttaagccttctataacattatggcctaaaaggttgttaaatagtaaaaaaagatggatgactaaagtccaagttcatgcttgggctaagtttatattgggtattttataccacgggttaacgggtatgggtgaaggcggaacgttctgattcccgtttacttattgggtgaagatttttgcctaataatagacctacgggtgaatatttatcccacatatatatcctagtggagtcaatatccatcggatatcggtcgtgggtacccattgccatctctagatcgaagagtagaaatttacttcctaaacctctctctgtctcatgcagcacaatagacgctttgtttcgttgcaacagcttgtttctctttgacgtccaaattcgtctatctacggacccacggccgcccagattttgaaatttcaaaacggaacacaccccggggttcggagtatctgctgcccctgcggtcctggaaagcccggcccacctctcacttgcaccaccagctcaccggttccggtcaacagtctctcgcgggtgcctgtgccggtggtcctccgtcctggctctggctgccacccacctcccgattaccgttctcgcctcgacttcaaaacaagagcccagatctaaaccaagcacgcccatctttgccacaccacacccccagtattcgaatctctcgtgcccagatgcggcaaattaaaaacaacggacagacgcggaacccctccggccaacggatctcaccctctgcggcatgggtcccactcacgctcgggtccactcgacagcgtgtagggcagagaggcgagcggtaccagtaccataggcctcccgacgcagtccgggcagcgggccccgcggattggaccggtcaaaaggcgtggcccaaccaaaccccaagggatccggcgctttgtctgcacgtgaatggtgccaagatcgcctggttgacaggtgggacccgtgaggttgtagacccacatgtctgtggcgttaaaggaggggggagggatcggcgggcgggtggtgcgcgcgggcaggcgggcgtcgcgtggtggtggtggtggtgggtgctttgactgcaggcctcggcagcaggcagagaggactagaggagtcggggcctcggaggaggggagggagagggcgaagagtagggggaaccaaatcttgaagggtaaacggagagttctttcgtggaggaggaagggggggacagcaggaggagggtagaggtatgtgcgcacccatctgttcttgctcctgatttggctgtttgttttttctgtctgttcttcgctgttggtagtttgtgaccgtgaatgggcgttcctggtccatgttcgcgtgcgctgctgccgattctgggagctctctggtcgtccgtctcgctgggatctgccttttccccggtgagagccgcggaacgttcgccgccttttcttactcgcgggccagttatggtttctggagcgttttctctgttcttggcgaggtggtcatcgctctgagaacgatgcgctctttctccgagtttgtgctcaagttttcgtcagcctagaggctatagcgtttgctgcggatctcacgacttctctcttcctcttctctattggtgcatacgttttcatccgaaatccattagttagtgcccgagccgtcaattctttgtggatttgcttgttccccttcgttacaggctcggaaatgcccctgaacagattcacaggggtcctagattaggattattttctatgactttccaagagtcaggagcacgattgctttctctcggctgtctgcctggttcatgactcagccgggtttgcaagcctaggaagaacttgctcacgtttcttacatttatctagattcgagggacgggttgtactcgttaacaaagttcacctcgttagtcattaaagctccgctgttgtgaatgatgctgccattgcgatatctggaatcatcgctctgatcgatttggttgttaatccacttacaggtagctcaatagatctactgctctcgggggagttaatgcaaagctgagttgctgcacgttggctttcttcagagatggcttcagctggtgtagccccatctgggtacaaaaacagcagcagcactagcattggtgccgagaagttgcaagatcagatgaacgagctaaagattagagatgataaggtgaagatgccttgatatcttgtttcgggcttactgtaatttcctcaagattatgtgaaaaatgggactgtgatgtaacctttggtgtgaatgccaaatgcaggaagttgaagcaaccataattaatgggaaagggactgaaactgggcacataattgtcaccactactggtggcaagaatggtcaaccaaaacaggtgagtgctttactgcatttgatcatgatttatcaactattctacatgtttttagtgcatgtctgaatctaataattgagagtcaagaccataatttaatgtccttcttttgcatattgccaatatatccatgttgctaacttataagattgtggagttgttctgatcagttttgtcagattctttttgtataataatgtgtatttattggttgcatttgcagacagtgagctacatggctgagcgcattgtaggtcaaggttcttttgggatcgtcttccaggttatttgcaataacttgtgactgactttgatatgtactattatgtagccgcctgtggtgttgctttccacggcgctgcacatgttttagatcttcatatcttgcgtgctataaatcacctttcttaatcagatgccatttcacctgttcataggctaagtgtttggagacgggtgagactgttgccataaagaaggttcttcaggataagcgttacaagaaccgcgagttgcagaccatgcgccttcttgaccaccctaatgttgttgctttgaagcattgcttcttttcaactaccgagaaggatgagctttatctgaacttggtccttgagtatgtgccggagacagttcatcgagttgtgaagcatcacaacaagatgaaccaacgcatgccacttatttatgtgaagctgtatatgtaccaggtaatggtttgtcctgttcctttttgctgttgttttaattataccttaaagcttatgttttgggccctgtttgatgttgaaactaacaaacatatttcatttcgcctaaatattgtctgctccaatgaatgtgctagttctttttcaatatttgatattatattggattttggcagatatgtagggcattggcttacattcatggcactattggtgtctgccacagagatattaagccacaaaaccttctggtatgctggaaaatctgctattttgctactgtatctttttgtaaagaaatgatttgtactttgaaattgatgttcaaacttcactacaggtgaacccacacacccaccagcttaaactatgtgactttggcagtgcaaaagttctggtcaagggggaaccaaacatatcgtacatctgctcccgatactatagggctccagagctcatatttggtgccactgagtataccacagcgattgacatttggtctgctggatgtgttcttgctgagcttatgctagggcaggtaaggtgtctcaaatttttattgccattttaaaaaaggttttcaagccaacaaggtcctttcagttcacactgtcttacaagaactatttggacagcctttgtttccgggtgaaagtggtgtggaccaacttgttgaaatcatcaaggtaattgtcggttctacaagcttgtgaattgtcttctatagaagcataaaatctgatcacccctaaaatgattttgtatggcaggtcctcggtacgccaacaagggaagaaattaaatgcatgaacccaaattacacagagtttnaagttcccnacaaatcaaangcacacccatggcacaaggtgcnnaaatctktctacattttgttacaatactctaagaaaanctgttactgttgnnnnnnnnnnnnnnnnnnnnnnnnnnnnnnnnnnnnnnnnnnnnnnnnnnnnntgttactwatttactttttgtacattttatctttcaggtmttccacaaaaggatgccgccagaagctgttgatctggtctctcggctactccagtactccccaaatctgagatgcactgctgtaagtgcatgccattgtacattatacatgatggaaatacccctgttgactttggttttctaagatcttyatgaatgttttgtccagatggaggcacttgttcacccattcttygatgagcytcgagatcctaatactcgccttccaaatggtcgctttttgccaccactattcaatttcaagcctcacggtatgtttcatgcctacataattcaacatcgttatcatagctgctacaaccaggtakcagtgtagtwcyaagtttgttctttgtatatcaccaccttacatgctcgccacctctgttctgcagaacttaaaggagtcccatcagacattgtcgcgaaattgattccagaacatgcaaagaagcaatgctcctatgttggnattgtgaaatgaccgcgccttgagactggaacctgtggttgcaattgtgaatttcccctgggatgtttgacgatctgaggcnatgcgagcctgttgttgaagatgcaaggttacgtacttgtacgacaatgtgacctgtgtagctgagtagtctatgtcgcagtgacatgtaacggcaccccccnnnttcctactaactgacgcttactcgagattgccatagttgatcttgtaatttgttatagagcagtatgaatgtatttatggtagcttgaatctatgtatggattcacttcgtttttccatgtttccttgtctccagacccagattgctaccgtattgtttcagaattcctagctacctgttgcctattgagtattgactaccagcttgcacttgtctgttattgcactggctgtggaatcagctgttgatttttgccacaatattttagttcagatgtactccctattctaaaaagaatgtgaaatcttactaatagaatagactactttttttagaatttctttccattttgaggaattaaaatcttactaatagaatagactacttttttttagaatgtgacattacaccactttctaaagttatcatataagcctatctcatttatggggtgagagatgaaaattgattatatagatttacatactgtttttccgatgtacaatttatagcacacccttctacttgcttcgctataacataaatgtagtatataactatctctttcatgtgatttaagataatatataaatatattacatatataaatatatgaacttaattagttttatctaaattataactattaaaataaaattcaatttcaacgaaacaaacggggccttgattaattataaaatgtatttttgtaataagttgatttaaagctataatgtaaatactatttactagaaacttggttaaatatgaattagtttaactaacgagtttaattggcataccacttatagttatattctttgagacggagggacgagtacgttgttcgatcggtctggaagtatgctgacttgatcgttcttaccagaaagttgcattattgcagcgtttgagacgactgacgaggaaatgtgacacgcagatgctactcagtgcttggcaggactgcattccaagtggtccttctggggagagaggaatcatagactgtagctccggtttcttgaaaaaaaacggttcccgtgaaatggcaggtatggttctccggttcctttgaaaactactctttgtaaaatgaagtatgcttggctctatcgaagttagctgttgttaacagccataccagacaggttctttcagtgtccggttagattttgaggcgtcgagggttgtttggttgagaagtggagagttcctttagagtgtgtttagttgagaagtggaggaaaatggatcgactatattcctattttttttatgtttagtttccaagaaaagcggagcagagcggctcctgaagttttagaaatttaccataaatagtttaaatgctcccgctccgtcaaaacgaacatacacgagcgctctcctccctctacttccttctacaaccgtatgtctttccaatcaagcaaagaacggagtagctctgctctattctactcttaaccaaacaaaaaaatgaagtgactctgttctgcttgtcaaatgcgaaatagaatgattctattctaaaaaattggaatagagccgctccaaccaaactaacctcactcgagggactaaagtttagtctttactctatttgattccaaggactaaaagtattcataacatattaaatgacttgaaaactaaaatgttcttaacattcttccgccattagcataactaaaataaactagggataagtgaaattaatatggactaaaacaatttggtcgctgttttattcccatatttgacaatttagaaattaaataaaactaaaatagatggattaatttttagttcctcaaacaattttttctaacaattttcgatggactaagtttagtcatttttcataagaaattaatatggactaagggcctgtttgtttacccctcagattatataatctggattaaataatcctaagaggcaaacaaacagtctagcttatttgtcgagattatataatctaactcctggattatgataatccataagcaagtgaggaggtgcttatttcagattatttttttccacttctccactaccctttcaagtttcctagaaattacccaccattgccattataacccaccattggcattcttgtcttcctcatacaa

SEQ ID NO: 8 - DNA, 570 bp, Zea mays
  misc_feature (217)..(477): r is a or g
aaggtgggaaaactgaaaaagacaatcatgaaggtgtaaattctttactatctgaggagttggaaaaactagctaatgggaatagcaaggtatgatataccctccatgattctgctttcatttattctttgttcatatggtatggttatttaacagtgctatgtattgccgtaaatgcagattcctggtacattagatgagtatagaaagcttgtcrttccaataattgaggagtattttagtacaggagatgtggaattggcagcttctgagctgaagtgtcttggatctgatcagtttcatcattactttgtgaagaagcttatatctatggcaatggatcgccatgacaaagaaaaagaaatggcatcgattctgttatcatctttrtatgctgatctactgagctcctacaggatcagtgaaggttttatgatgcttctggagtctacagaagatctaactgttgatataccrgatgctactgatgtattggcagtttttattgcacgggctattgttgatgaaattttgcctcctgttttcctcactcgagctagggcactactt

SEQ ID NO: 9 - DNA, 501 bp, Zea mays
  misc_feature (7)..(478): n is a, c, g, or t
  misc_feature (292)..(292): m is a or c
cggtttnnnggccnancnncatatcccacgtttgctggntgaattgtctggccttgagaagttacttgntgcaactggcccagttccagacccatggcatcatttgcagaccctgtcagcatgttaggtggtaagaacgaaaangtgtcatcatatggtgcctggacattggnggatgaactctgcagctgagatggatgtgttgcgctttggtcgangccataccctgcagaatcagttccanctgaaaaaaaattatagagagcactgcattcaaanttcaaaggctcamtatactgaagtagcatatttacatatcntaaagccttgtatcaaactaaantatcnatatcaatgtacttacaacaacaattagggttnnccagttnaacataagctacaaactgaaacnntcaagataatagagctnnnnntnnaattgtatctgngcctcagatgctgctcacctgatggtganggccctggcatgctcatcgaaga

SEQ ID NO: 10 - DNA, 1260 bp, Zea mays
  misc_feature (166)..(166): r is a or g
  misc_feature (205)..(1251): n is a, c, g, or t
cacgccgacttcagtaggcgaggcagggtgtcgtcgcttcatgcatgcgctggcattgcttctcggagcattcgcagccattcctacaggtatagactatacctatacgtgcatgcgcatccatccacccataatccgtgcatgcatgcatgattattgacactartgtccttattactaaacaggagtccaatccatcggcgtntgctacggcgtgaacggcgacaacctgcccccggcgagcgacgtggtgcagctgtaccagtccaacggcatcaacctgatgcgcatctacttcccggacgcnaacgcgctgaacgcgntgagcggcaccagcatcgggctcatcatggacgtgcccaacacggacctngcctcgctggcctccgacccgagcgcggcggccgcctgggtgcagagcaacgtgcaggcgttcccgtcggtcagcttccgctacatcgccgtgggcaacgaggnctccggcggggacaccggcagcatccttcccgccatgcagaacctcaacgcggcgctggccaacgccggcctgggcggcagcatcaaggtgtccacggcggtgcagagcgncgtcacccagggcttcccgccgtcncagggcaccttctcgcagggctacatggcgcccatcgcgcagtacctgcagagcaccggcgccccnctgctgtgcaacgtctacccctacttctcctacntcggcaacccggcccagatcgacctcagctacgcgctcttcacctcgccgggcaccgtcgtgcaggacggcagcaacgcgtaccagaacctcttcgacgcgctcgtcgacaccttcgtctccgcgctcnagaacgccggcgcnggcaacgtcccngtcgtcgtgtccgagagcggctggccgtccgccgggggcgacgccgccaccgcggccaacgcgcagacctacaaccagaacctcatcaaccacgtcgnccagggcacgcccaagcgccctggccccatcgagacctacatcttcgccatgttcaacgaggaccagaagacgggagccgagtcggagaggcacttcggnctcttcaacccggacaaatcgccggcgtaccccatcaatttctcctaattcctaaacaagacgccgaggtccattccaagacatttataaggcaatacacacacatagatatatatatacacatacatacgggggaaaactgaataaataaacgcctgaagtataagcatagagccnnnnannnntcggacccc

SEQ ID NO: 11 - DNA, 522 bp, Zea mays
  misc_feature (139)..(454): n is a, c, g, or t
  misc_feature (148)..(148): k is g or t
aaggactttggaggagatactctatgctctggttgttcagaagttcgttgaagctggtgtctctctggttccagcactctcacgctccaccgatccttctggaagagttgatcagtgggcagaaactgtggaagaaaancttcaacgkctgcactcgcangaggcctatgaaatgatcgagaatcacctcaccctcatnctggggcagcgtcaaggtgacgccactatcgcagccataagtaagctccgngttggccaggtctatgctgcatctgtgatgtacggttatttcctgaagagagttgaccagaggttccagctcgagaagacaatgaagggcctcccttggggntcagaagaggaagacagcgctttgaatcaagttatgatgaccgacttgatgccttcagctcagacttctagctctcatccagagatgggctcgtggaccgcncctgccttcagcacaggagggcccagccaatctatcaagccttgccgccttaggtcgtatgtcatgtc

SEQ ID NO: 12 - DNA, 157 bp, Zea mays
  misc_feature (34)..(34): n is a, c, g, or t
  misc_feature (94)..(94): s is c or g
gtagtccttgagcgaccagaagctgatcagcgcngtggccgccatggcgacgcagaccatgaagttgctcgtcacccacaccaccctcggcccsaccttccggcacatgggctcgatcaggaacgagctgaatcctagaacgatctgcacgtacggt

SEQ ID NO: 13 - DNA, 145 bp, Zea mays
  misc_feature (35)..(35): w is a or t
  misc_feature (86)..(86): m is a or c
  misc_feature (89)..(89): s is c or g
  misc_feature (116)..(120): n is a, c, g, or t
atctcaccgagttgagcagcagcccgaacgagccwactctgacgccttcgtcgaacgcggtgtcgtagaggatgaacgggaaccamgasagctgcatggacgacacagtgcatggnnnnncagcagcgtcagccgtcagtaaaga

SEQ ID NO: 14 - DNA, 736 bp, Zea mays
  misc_feature (63)..(681): n is a, c, g, or t
  misc_feature (432)..(432): r is a or g
tgcaagaagcacactctccacaaggttactcagtacaagaagggtaaggatagcctgtctgcncagggaaagcgccgttatgaccgcaagcagtcaggatanggtggccagaccaagcctgtcttccacaagaaggtaatgaagtatacctatgtgattgtactattgctccatcaatccttcatctttgtccgttttgatgctagcatgaaagactgaaaataacnnncatttctaaatgtctgttnnnnnnnnnnnnnnnnnnnnnnnnnnnnnnnnnnnnnnnnnnnnnnnnnnnnnnnnnnnnnnnnnnnnnnnnnnnnnnnnnnnnnnnnnnnnnnnnnnnnnnnnnnnnnnnnnnnnnnnngggtgcacagattgggatatgacaaatgttgtgattttcaggccaagaccaccaagaaaatcgtrttgaagctgcagtgccagagctgcaagcactactcacagcacgcaattaaggtgcagtgtctcattttcctgtgttaggcttgctgttgcacnaagtattgtctcactttgatttagctcactctttcctgactgactcncctgtgtcacagaggtgcaagcattttgagattggtggaganaagaagggcaagggaacatctctcttctaagtttctcatcgcncatctcgatgttggatcgaanctntgggtctactactgttctaaaaactcgtcaaatttcaatgttactagtagttctg

SEQ ID NO: 15 - DNA, 835 bp, Zea mays
  misc_feature (27)..(826): n is a, c, g, or t
  misc_feature (753)..(753): r is a or g
gagaagacctgctccttctttgtcggnatggtggtgttcctggggatgagcacagtcatgacgcctccngccgtctccaggccgagcgagagcggcgagacgtcgagcaggagcagatcctgaaccttctcnttgccctcgccagtgaggatggcggcctggacggccgcnccgtacgcgacagcctcgtctgggttgatgctcttgcacanctccttgccgttgaagaagtcctggagcagctgctgcacgcgggggatgcgagtgganccgcccacgagaacgacgtcgtgcacgctgctcttgtccatcttggcgtcgcggaggcacttctccacgggctccatgcacttgcggaagaggtccatgttgagctcctcgaaccgngcacgggtgatggtcgtgtagaagtcgatgccctcatagagcgagtcgatctcgatggtggtttgggcggtggaggagagcgtcctcttagccctctcgcaggcggtcctcagncgccggagcgccctggggttgccagtgatntccttcttgttcttcctcttgaactcctggacgaagtggttcacgagccggttgtcgaantcctcgcctcccagntgggtntcgccggcggtggccttgacctcaaagatgccctcctcgatggtgaggagcgagacgtcaaaggtaccgccgccgaggtcgaagatgaggacgttcttctcgccgtcgctgctcganttcttgtcgagcccgtatgcgatrgccgcggcggtgggctcgttgatgatgcgcatgacgttaggccggagatgacgccggcgtccttggtggncnngcgctggga

SEQ ID NO: 16 - DNA, 1024 bp, Zea mays
  misc_feature (23)..(967): n is a, c, g, or t
  misc_feature (755)..(755): y is c or t
tatagtacgttttattcgacacnnnagcctctgcatgcaataatagtacancccccgatttaattaattggactaatgcatgctgaggatngatcagatggagatgctgctggggatgcccctcccggtgactcccggcttggagaagggcttgagcagctcgtacggcacgatcccggcgccgcagcggttcttgaggtccaggttgttgttgcactcgtcgatgaacccctcgatctccttcatcctgccgccgaacttctcgaacgccgccttcaccatgggctccgccagccacganggctccgcgaactcccccatgtactcctcgtcgggcgagngcgacgagaggatgtccagcgtcgtcatgaccttgatggcctgcatctgcgngggcagcatgtccagcagcgtcgtctccggctgcttgaggaacttctccatctccncgcccgncccgccctcctccaccggcatgttcttccggatggtggtcggccggttggggaagtagccggcgaagtggtactgnccgaagttgacggccgagtggtggccggaggtgacccacatgatggtggtcagcgtctccaccaggctgtcgcgggtgtccagcacgggccaccacggctcgtccttcttgtcgccgtgccccacgttgcgcacctcgtcccagaacgccctcagctcggggtcggcggccacggcctcgtcggacttgtagtagacgttgacgtactcggacgcccactgcytgatggagtcccagaccaggagcccgtcgtgggcgtaggggtagtccttgatggtgagctccagctccccgtcctccccgcgcacggccagcccgcgcttgangaggtcgttgggcagcgcctccgtgtcgaactgccacgtcgcgccgtacgccacggagctnagntcgacggcgtacttncccggccnnnangnnnncnnnnnnnnnncntcggcgttgatgagcgcctccctggccagcgcgttgatctccatggtgtagcggaag

SEQ ID NO: 17 - DNA, 499 bp, Zea mays
  misc_feature (222)..(222): n is a, c, g, or t
  misc_feature (431)..(431): s is c or g
gacaagctcgccatactgggtctcccgatctggattactgagttggatgtcacagcagagaacgagcacatacgagctgatgatctagaggtgttcctccgggaagcatttgcacatcctgctgtggggggaatcatcctctggggattctgggagatgtttatgtttcgagagcacgcccatctggtcgatgctgatgggacaatcaacgaggctggcagnaggtaccttgctctcaaacaagagtggctgacccgtatgaacggcagtgtcgatcaccaaggagagtttaagttcagaggataccatggttcgtacacagtggaagtgaacacgccttcaggcaaggtagctagatcgtttgttgttgacaaggatagcccggttcaggtgatcgctctgaatgtttaatgtgtgggaaatcatgcgcstgtcctgtattttagcgatgtactgaggtgttgaacacagatagtttcatagctgatgccacgccttc

SEQ ID NO: 18 - DNA, 886 bp, Zea mays
  misc_feature (32)..(883): n is a, c, g, or t
  misc_feature (518)..(518): k is g or t
gtcagtagttcatccatttgtcccattttttnagcnnggaagtttggttncactnnncttggtctaataactgagtagtcattttatnacgntgtttngacaagtcngtagctcatccatctgtcccatttttttcngctaggaagtttggttncactggncttggnctaataactgantagtcattttattacnttgtttcgacaagtcantagctcatccatctgtcccatttttcagctaggaagttcggttgcactgaatttgtgaacccaaangaccacaacaagccngtgcaggaggtctgtntctttacccaagncaacaaaaggttatcacagcttatgctgaacttggccataacattcaataattcctttatggtctaggtacttgctgagatgaccaacggaggggtcgaccgcagngtggaatgcactggcaacatnaatgctatgatccaagctttcgaatgtgttcatgatgtaagtatatgtatacactctcagctactttckttctccaggttcccttcatccagacatgcatgttctaacngccgcnctcgtgatccagggctggggtgttgcngtgctggtgggtgtgccncataaggacgctgagttcaagacccacccgatgaacttcctgaacgaaaggaccctgaaggggaccttctttggcaactanaagccacgcactgatctgccaaatgtggtggagctgtacatgaaaaaggtaaattgcaaagtgcngttccttcngtttccttaccngccgagcttttngctgaaaaactgttaagaatcgttcctgcaattctgnnnnnnnnnnacaggagctggaggtggagaagttcatcacgcacagcgtcccgttcgcngag

SEQ ID NO: 19 - DNA, 904 bp, Zea mays
  misc_feature (87)..(842): n is a, c, g, or t
  misc_feature (182)..(330): r is a or g
  misc_feature (463)..(463): s is c or g
atgcgcccttgggtacatagcaggagactggaaaggtaacaaatggaatacggacacgtagataaccatggaggcccagcaatgttnnngaggnnnntattgtttggtcactgcatagccgatgatgatcaccacgcnctcgtgnatgcctcatgtcttaacagcagccagatgatctctgrgcccggttgccacctaccacatccacggtatctggcacataccttcaagaacaaatcgataaggtcaaaaaaaannggggnacggcttttacatagataataaaggaccagcacagggaaacaaatraaggaaatcnaaaagtgattratgattttacatagatataacactgaaaacgagaccagcagaagaagctagtcttattgcagcagctaatgatgccaaccctggtacacccccnagaaagaggatcaacannnngaanagnnnnnnnnntngsnncttattttgctgatgactaacaactggangcaaaaagaccaacagaaggaccggttgatattaaaaatgtaattacttttancagcnagcgnctccggttttctagtacttgcagcaactaatgtcacataaaaacnnnnnntgtcaaatgccaatcaaacacacaaannnngaaacgaganatcannnagngntgtgcnttacaattcttcctccnggttcattncnttcagagcattctttacaatacactggaaggcatcttccacgttcgttccatnccttagcagacgtctcaaagtacgggatgttccctttagaggcgcaccatgcctttgccntttttctccgacacctaaaaccaaagcagattatantttctaagcagctcgtgatccagttcaagagaagaatttattcagagaacaaatcatgtagc

SEQ ID NO: 20 - DNA, 815 bp, Zea mays
  misc_feature (52)..(438): k is g or t
  misc_feature (96)..(96): r is a or g
  misc_feature (152)..(296): y is c or t
  misc_feature (180)..(180): w is a or t
  misc_feature (208)..(208): m is a or c
  misc_feature (419)..(419): s is c or g
  misc_feature (773)..(776): nnnn is ctgg or gtgc
ggtttgtctgtttcatgaataatgttctgttgcgtcaaattaatagcaagtktctgatatttttttttctccagcatgtttttgaatactttacaraaagaaccccaagatcccatttcgaacatcgkgaaacatcatttgtgtggaactayaagtatgctggtaagtgtttatcttccwaacattctttttaagcraggtctgtgcmgtaacattttatttccaccttctatytcaaagatgttgagttyggaaggctacaagcaagagatatgctgcagcacytgkggacrggyccgatctcaaatgcagctgttgatgttkttcaagggagtcgatcagttgaagttcggtctgttggagttaccaaggtaagtggtgctgtatgatggtccatgacagtagatggtttgrcctasttgaggttttaaacatcakttgtctccttcctatagggtgctgcaattgatcgtattttaggggagatagttcacagcgaaaacatgattactccaattgactatgtcctgtgcatagggcatttccttgggaaggtaatttccaattcttcacgttattgttctgatctggttttagttctgtggataggatcaagaaacttatgaatgaagaratgraagggtttagaacattcaaaatgcattgccaaggaaaggagaaggatgtggacttaattagaaaaatcactatggtttactttatatgtttggtctgtccctattcttttcgactttggtctgttttgtaacatnnnnttcctcgtgtttcagratgaggacatctacgtcttcttt

SEQ ID NO: 21 - DNA, 426 bp, Zea mays
  misc_feature (61)..(200): y is c or t
  misc_feature (310)..(407): n is a, c, g, or t
  misc_feature (316)..(324): nnnnnnnnn is gcgtacgtg or is absent
tcttcagtctccaccctgattcaacaacagactctgacagcttgcacggtagctgccccgycatcgaaggccagaagtggtccgcgactaaatggatccatgtgaggtcatttgacctcaccgtcaagcagccgggtccctctgatggatgtgaggacgacaatgtcctctgcccccagtgggcggccgtgggcgagtgygccaagaaccctaactacatggtggggaccaaggaagcacctggcttctgccggaagagctgcaaagtatgcgcagagtaaggtatcggtcctctgcgtctgatgagtantcgtgnnnnnnnnnttacgtagttgctgtcaccatttnaccagggtttagatacgaccgagtacagcatgtataagacagtacaancccggaagnnngagtcgtaagagttagggg

SEQ ID NO: 22 - DNA, 432 bp, Zea mays
  misc_feature (1)..(432): b is c or g or t
  misc_feature (1)..(432): k is g or t
  misc_feature (1)..(432): m is a or c
  misc_feature (1)..(432): r is a or g
  misc_feature (1)..(432): s is c or g
  misc_feature (1)..(432): y is c or t
  misc_feature (265)..(375): n is a, c, g, or t
graagcgaacgaggaaaggaagaacaagttggctycgatygaaggckcracaactgccgagtaccatctgcctgttctggcaatgacagcygatgttatmcaggcaacttaygaagagtgcataaaatcgggaatggayggrtacgtatctaaacccttcgacgaggagcagctataccaagcagtctccagattggtagtgggaacgacrgattcggctgtttgatgttcaaaatacgatgsmmcbgacttctcattcrtcgannnnagtgaagcatcaccatmttgcmtctgtccagctgactctanntcccttgacaatgggcctnngacatggcctctcacaagactagatgaaaaaannnngaagatnnngaaagtgccgtgagttagstacgyrtcacacatgacatgaagttgctgcggcagccc

SEQ ID NO: 23 - DNA, 880 bp, Zea mays
  misc_feature (116)..(217): r is a or g
  misc_feature (515)..(856): n is a, c, g, or t
attttgatccgtcattatcttgctcaaattctgtaactttcatcccaaagttcgccagaattcgtttcttttttattttgttaccagtagagcatctcctgatctacctcttcgtrgtgtttggtaaagactattgagctcaggtgtgttgcgttgtgcagagcacaagtggtgggatggccaccagtctgcaactaccgcaagaacacgatgactrccacccagctgaagggcagcaaggaggatggtgatgccaagcagggtcaggggttcctgtacgtcaaggtcagcatggatggcgcgccgtacctcaggaagatcgacctcaagacttacaagaactacaaggacctgtcgaccgcgcttgagaagatgttcagtggcttcagtactggtgagatgtctcggggttactctctctctctctctctctctctctctcggatggcgcgacagagagtaattatgtttcgttttgatgtggatggtgatagaagcacatcaagaagtctttnaaaaagcagcatactcctacttgattcctaggataagcaatagcttgaacttaccccgatatattttgagtaattgtgagattacacacaatctggcacgccttgttttgttaatttttgggagaactttatatttctcccaaaacaaataccctggagattgttcagatattgcatccgtatcaagtctctcttagagagatgtagttttctgtaaggcaaaataagttgtgtctccatctatatgaatatgcgaggatatcttcgagctctgagtatnattccatagagagctactaatctctatgagagtgacctccccntatatattcctgaaattnttggagatctgcggccctgtatat

SEQ ID NO: 24 - DNA, 921 bp, Zea mays
  misc_feature (106)..(913): n is a, c, g, or t
  misc_feature (746)..(746): m is a or c
cgctgaatccaacctaatgctgtacagaatatcctttacagccaagccgccaaccaagacgctgagtctaatgccatgtcctggtggatccaactatccaaacaancagatcaccccctttgagctgactgacgatcatgatgctgaaagtattggatgctggtcgaaggcttcaccctcttgctggctgtgaagtggaagacagagtcatgtaatcagtttgcttgccttcaaatcatacacctggtgtaaagtacagtttggtttgaatataaacaagtatcataaagtacttctttaaaattgtccaacgggggagtcagctgtcttttgcacctcagggtgcttcacacgtagctatatgatggtcactggttaactcatttacatagacaatttcagaagggataatctatgcaaaatctaatgatattattatgacccctgatccatttagaacaacatgagctgtactcctcctagatatgattacataagcatcttganntctatcaggcctttggtgagtactcaacactcaacagaaacctactaactcctatcgttctctgattaaacgagtgaacagttcaggacactgcagaagatttttttttnctataagccaccgctattcaacaatcaacggnttttgctaatcagatgtcacaaatgccaacatattgtcatccgaggatattccgtaaggtggacaagatagaaccagnttatctcagaaaaaaagmccattaaaggatatctggtaataactacatcaccatccttctgtattcaagtattagcagaagaganttgataatggaaggaaatcatccctgaantaagcaccagtaatngggnatatggtcatgntatcaaatgtaatttattaagcatcgcaagttttagaatntagcaacc

SEQ ID NO: 25 - DNA, 831 bp, Zea mays
  misc_feature (42)..(633): n is a, c, g, or t
  misc_feature (562)..(562): r is a or g
acaaaggaaagggaaagaaaatgacttctaggttttcacgtnctccttttggttgaccaagaagagatggtcggtagagtgaatggccttgtgccatctcaattctttcgcgtggatcatacattgtctcatctcttatagcctgaagaatcgaatcagcaggacggtccctgtgcacatatatgtaaacagaccaactcagtcaaatatcataaaaccttagttcaatgaattatttccaaactattggaagataaagtagaatagctggcacacatgcaggggcagaaggaaccatgccaatcaagttatcggtatgtatgggttagtaatataggttactggcatnnaggtaatacgctgaaaatgtaactggtgtagagtatgtggcgttggtcttaggttctaacctcgtgatcagaatcctatgtagtgcttttaggatcgggcacatctcaaccggcgcaacagatctgttggcttctggatgcatgacacttaagctatcctgactaagaagctcataaaacgcatcaactgcagagacaccctgaaatggaarggcaacaggntaattcatcacatgattcatttaggcatattcatgcagttctttgaagtttcgttgtcgancaaaattaaaagggcatacctgaatggtcccttttcctttaatactgtcacccatttctaatgtcaattcacctttagctaacttctgcccataccatgcattacgacctttcaacaatgtgacataagtgtcagctaataagggtccagcaagtttttcaggttcttcttccagaaggtgtgtgatgtagatcatct

SEQ ID NO: 26 - DNA, 1901 bp, Zea mays
  misc_feature (687)..(1892): n is a, c, g, or t
  misc_feature (1271)..(1271): m is a or c
taccttgtttccccaccagagatagatagaacatctggggagtacttggtgaagaatggcatccgcacctttgcttgcaggcaagtactatctatttctcagcctttctcttgatacttttttatttacttcaatatcgtaaaatcacttagtttttctgagtcatctaagtcagcatgctccatttattttgaatcaacattatcaagtgtacttcgtacaatcttgtacatacctgtgaggagcactgaccttctggaaagatatcatttttcacttcacagaacatcaggaattcaagattcactcagttaattgatattttaaataattttgaaaattgaaatacaggaaaatatgtgtttttaaggcattacattttgcatataaatattcaatctcactaaaggaaaatgttttaagaacatttttctttagtgaaaaggaatccaaatgctttcgaattctgttgtgacttatctctattaccttatactgcatccgtactagtatatttgacatctgtagagaagagttcttttttctagggtaatcttctagctgcagtgcagtatgctgacattgtgctaacttaggctgatatttggttgcattgctctgcccatgatttgtgccctaatactgtatattagggctgcataatgttatttttggattgattcattnnnnnnnnnnnnnnnnnnnnnnnnnnnnnnnnnnnnnnnnnnnnnnnnnnnnnnnnnnnnnnnnnnnnnnnnnnnnnnnnnnnnnnnnnnnnnnnnnnnnnnnnnnnnnnnnnnnnnnnnnnnnnnnnnnnnnnnnnnnnnnnnnnnnnnnnnnnnnnnnnnnnnnnnnnnnnnnnnnnnnnnnnnnnnnnnnnnnnnnnnnnnnnnnnnnnnnnnnnnnnnnnnnnnnnnnnnnnnnnnnnnnnnnnnnnnnnnnnnnnnnnnnnnnnnnnnnnnnnnnnnnnnnnnnnnnnnnnnnnnnnnnnnnnnnnnnnnnnnnnnnnnnnnnnnnnnnnnnnnnnnnnnnnnnnnnnnnnnnnnnnnnnnnnnnnnnnnnnnnnnnnnnnnnnnnnnnnnnnnnnnnnnaaatggtgacatggttggtcacactggtgatattgaggccaccgtagnttgcttgcnaaggcagctgatgaagctgttaaggtgagagcaccaatgaaagttcgctgacatgtgtgttgtcttattatctgcattggaagttcgcttatacatcaataaaggttcttacagtagcacgcmtcataggcctttgcctattttttaaccaagtgttcttctgaacagattattttggatgctgtcgagcaagttggtggtatttaccttgttaccgccgatcatggcaatgctgaggatatggtgaaaaggaacaagtctggcaagccgttgctcgacaagaatgaccgtatccagattcttacctcgcatacccttcagccggtgagtgcaatgccatttgaccccatgtcttttggttnnctctcccagcaaaatcatacccgtgttgattgcttggatgctaatgcctctgtaaaacttgcaggtcccggttgccattggaggccctggccttcaccctggagtgaaattccggaacgacatccaaacccctgggctcgccaacgtagccgcaaccgtgatgaacctccacggatttgaggctcctgctgactacgagcaaaccctcattgaagtggctgacaactaaacactggccacctgtgtccaattttggttatatgtagttctgagaatggacattcaataatttatgtttgcaagcacgttgctcaaactcaccaaaacatcgagggatgccttttgactttggcatttacagcattttcgtttggctttaanccttatcgg

SEQ ID NO: 27 - DNA, 595 bp, Zea mays
  misc_feature (64)..(64): s is c or g
  misc_feature (201)..(576): n is a, c, g, or t
  misc_feature (254)..(254): y is c or t
cgtccgcggcagcggccgcgtccaggtggtcgggcccgacggggtgcgcgtcctggagacgcgsgtcgagggcggcttcctcttcatcgtgccccgcttccacgtcgtctccaagatcgccgacgcgtccggcatggagtggttctccatcatcaccacccccaagtaatttgttgtctcgatcgatcgatccatcgatcnnnntttttttattgcgaattgcactggagatttgattgcacgtgaattaatgyttgcattgcattgcagcccgatcttcagccacctggccgggaagacgtcggtgtggaaggccatctcggcggaggtgctgcaggcgtcgttcaacaccacgccggagatggagaagctgttccggtccaagaggctcgactcggagatcttcttcgctcccccatccaactgagaaaataggccggaagccccacggtggagtnnnncctctcgttaggtcgtcgtgcttagattaggttagctagcttgcctttaataaaaagagagtggtggtcgtcggcgtcggcttcggcggtctgcttcttcttcattcnnnnnnnnagtgcgtcggtcggtttag

SEQ ID NO: 28 - DNA, 558 bp, Zea mays
  misc_feature (39)..(550): n is a, c, g, or t
  misc_feature (98)..(496): y is c or t
  misc_feature (224)..(224): m is a or c
ccgtgttggttggatctatggctcggtgacggaggatgntggtcactgggtaccggantngcacaanccggggttggaangntcggtgtactgtgtnyaccaangcgtgancgccnttccgcggcaccgcgcccatcnaacctgacyganccgtncntnccaccanggtgcntnccggtgggctanctggnantcnagtggagantcnttcnttncntncccgmaacnaancngcgctgctggcgangccgcagnaantgnaagnttcttgcagaggnantcgcgtacctgnaacgtgggtatctacccgttcacgtccantncttccntngatncgtctactgcttncctgccggcgctgtcgctgttnctcggggcagttcatcgtgaagnancgctgaancgtgacgttncctgacgtacctgctggtngatcacgctgacgcntgtgcctgctggcggtgctnggagnantcnaagtggtcggggatcangyctggaggangtnggtggcggaacgagcagnttnctggctgatcggcggcacgangcgcgcac

SEQ ID NO: 29 - DNA, 937 bp, Zea mays
  misc_feature (92)..(668): n is a, c, g, or t
  misc_feature (258)..(258): y is c or t
aatgtgatatcatgatactcatgcacctgtaccttagccaatgcaggagtctgttaaagtctcaataacattttgtgatgctcaccaacagnttcctttttacaggattcatctggtatattctgggataatgacagtttagctggtcttttggctattgaacttaaagcagatctccttgttctactaagtgatgtagatggtctatacagcggtccaccaagcgaaccgggatcaaagatcattcatacctacatyaaagataaacattacagtggaataacttttggggataagtcacgtgtaggtagaggaggaatgacagctaaagtganagngctgcttttgtggcttcgaacagtggcacacctgttgttattacaaggtatgtattgcatttttcattctttatncgagaattaaaactgcccttcgttgctcatttatatgttcccatgtgattgtgatctatcaaactttccctgtgacatgcaaccaataataaggaatttagacaaaacagttgataggtggtgtgattaactacatatttggtgtatactacatttgactcaagtgttttatttttggnnnnnnngtgtagactacatttgactcgagtgtttcttacatctttaatgatatgaagaattggttttcagaagtgnaaatatttccttagacttttttctctctcgaacgcgcaggagagctgcacatcattatatttccttagactgttatgctgaatcctcgcttgtgatgttcacttatttttctatgttggattttatttacatataataaggtctgttggtcaaatccaaatacgccatctgttttcaatgtttgttcacggccttaggaaaatgtgttgcacattgtttgtctattgaggatatcaggagtgtagttattgctatgtttccactctccc

SEQ ID NO: 30 - DNA, 1193 bp, Zea mays
  misc_feature (8)..(1108): n is a, c, g, or t
  misc_feature (259)..(259): y is c or t
  misc_feature (296)..(296): w is a or t
  misc_feature (398)..(398): r is a or g
  misc_feature (1057)..(1057): s is c or g
gtgaatgnacagggngactcctggnacagcctactcggcaggaacaagcacgacgaccaggagaagaagaaccagcagnnnnnnnngncggaggaggagnnnctggcgaccggcatggagaagnnngtcacggtnggccgagcccgaccacaaggaggagggacacgaggccgccgagaagaaggacagccttctcgccaagctgcaccgcaccagctccagttccagctcggtgagtnnnntcgtcgtaaaacatgayctgctgctagctagtttaattgactccgccttcggawcagtaagctaataaaccggcttctcactgcgatcgtggtgcctgcgcgcatgcagtcgagncgacgacnaggaagaggaggtngatcgatgagaacggcgarattgtcaagaggaagaagaagaagaagggccttaaggagaaggtcaaggagaagctggcggcccacaaggcnccacgatgagggcgaccaccaccagnnnnnnnnacnngcccnngcgccnnnnnngcccgtggtggtggacacgcatgctcaccaccaggagggagagcacnnnnnnnnnttcccggcgccggcgcctcccccgcacgtggagacgcaccaccnnnccgtcgtcgtccacaagatcgaggacgacgacacgaagattcagnaccccaccacaggcaccggangaggagaagaaaggcctgctggacaagatcaaggagaagcttcccggtggccacaagaagccggaagacgctgctgccgccgccgccgcgccggccgtccacgcgccaccgccgnnngcgccgcacgccgaggtcgacgtcagcagcccncgatgnngncaagaagggcttgctgggcaagatcatggacaagataccccgctaccacaagagctcgggtgaagaagaccgcaaggacgccgccggcgagcacaagaccagctcctaaggtcgcagnnnnnnnncgtgtgcgtgtccgtcgtacgttctggccggccgggccttnnngggcgcgcgatcagaagcgttgcgttggcgtgtgtgtgsttctggtttgctttaattttaccaangtttgtttcaaggtggatcgcgtgngtcaaggtccgtgtgctttaaagacccaccggcactggcagtgagtgttgctgcttgtgtaggctttggtacgtatgggctttat

SEQ ID NO: 31 - DNA, 482 bp, Zea mays
  misc_feature (121)..(471): n is a, c, g, or t
  misc_feature (239)..(239): r is a or g
gcaaaggtacagcgtaaaaactaagaggagagccagcaagctagcattttatttagtaaaatcgttcactcgcaggtacccaatcttctcagctttacacactcgccatcttgaggctgtngcccttctcctgcaggctcacgagtaggcngncaaagctcttcttgaaggagtccangccttccagctcaagctgctttccnacctcnncccagncnatgccaagcttctccaaggcrctgtatacaccttccgcctcagacacnttngcatcnactgtcctnganacngtgccgtggtctatgaatgcntgcaaagcttggtcgggcatcgtgttgacctgaaangtgcancannnctacagagttattttttnnnnnatgataagaaacaangccanttcaagtggnnaactcgtcgtgnnancatnccgtgtcaggtccnatgagactgtcnanntaaagagtgtcnggataagctgg

SEQ ID NO: 32 - DNA, 376 bp, Zea mays
  misc_feature (12)..(355): n is a, c, g, or t
  misc_feature (208)..(208): r is a or g
ccaggcgaccanggggttcaagaacaagatgctgctcggcnccggcggcttngggagggtgtacaagggcgtgctcnccgggtccaagctcnaggtcgccgtgaagagggtgtcgcacgactcgaagcaggggatgaaggagttcatcgcggaggtggtgagcatcggccacctccgccaccggaacctggtgcagctgctgggctartgccggcggaagggcgagctgctgctggtgtacgactacatgtccaacggcagcctggacaagtacctctacgacgncaggaccgccaggcccgtcctggactgggngcagaggttccagatcgncaggggcgtcgccgccggcctnctgtacctgcacgaggactgg

SEQ ID NO: 33 - DNA, 839 bp, Zea mays
  misc_feature (346)..(837): n is a, c, g, or t
  misc_feature (391)..(391): r is a or g
aaacaacaacttgttgttgtccacaacaggttaacagatcaaagaaggataggtgagcggcactactcatctcgtggcttctggatctggtgacagatgatcagcccacgaaggaaaaagaaaaagggactcgcttgatttgcgttgctttgctttccgcgcaaggccgaaagcttaaggtcggggcaacgagtacaccgagagcgacggagatatatcacgctctgctgcttcatgatagctggaaggacatcagcatgacacgcatgccaataatgtagtagaagactagtttatttgtcacctactaggcagagagtgcggtggttccatgaaccaaccattnnnncgtgcgtgcgtgcccaccgcacgaccacgagggggcatgcarcatatactttacaaaattcattcggttgttgacttggtttcaattcattgggttgggaagacaaaactaacatggatgcgttgcgtactcacaggaaggtgatggctcagactggtgagatccggtgcgccatggatcacatcctcgaggccgagaggaagggcgagatcaaccacgacaacgtcctctacatcgtcgagaacatcaacgtcgcaggtatcgnnnnataatcgtcactgctcagtgcaatgaaacggaaacagagtatgctatgtctgaagaaccaagtgagnacttatcattcaactactgcagtccagcgctactacacaaacaaatagcactgcaatatcggaagatataataatataaggcacgtcttaatcaagtctccgtcagccaacttaattccntccttaattaaccggcaacatactgagcctaangc

SEQ ID NO: 34 - DNA, 693 bp, Zea mays
  misc_feature (145)..(146): nn is ca or both nucleotides are absent
  misc_feature (169)..(169): w is a or t
  misc_feature (174)..(590): n is a, c, g, or t
  misc_feature (537)..(537): w is a or t
tgacctacaactcaaacaggctcgtcttcaatggccacgagatctacccgtcagcagtcgtgtctaaaccaagagtagaggttcaagggggtgacttgcggtcgttcttcacattggttagcaccagtccaacactactccacanngttagctctccaagttgttctawatatnnnnnnntgtatccnnnnnnnncttcctttccctaatggccatagttcctgaatntccaggttatgacagacccagacgtcccaggaccaagcgatccatatntnagggagcaccttcactggtaacatctggcatttcctaccaanncatctaggggaatgctgtgtgactgnnatatgtcctttacatttgcaggatcgtgactganatacctgggacaactgatgcctcattcggtagtnnnnncncccncctctgctttgtggttaattagtngttccagttgttcttgnanctagtnaattnnnancaggcatttntttttcagggagagaagtcgtaagctatgagagcccgagaccwggcattggtatccacaggttcatctttgttctcttcaagcagannnagcgcangcagcagcagactgtagcggcggtgccatcctccagcagggaccatttcatcacgcgtcagttcgctgcggaaaacgatcttggccaccctgtagccgctgtg

SEQ ID NO: 35 - DNA, 765 bp, Zea mays
  misc_feature (76)..(76): r is a or g
  misc_feature (97)..(625): n is a, c, g, or t
tatgcatgatttatgcccgccaaacagacagaaaacgcaacaaactacaaccatttacagaccggagccaagtgarcctaacttgttaacatcatangaaggnacatcctaaacgagcaatgcttactcaaatttactgctatgctacttctattgctgttaatgaggcagtcactcacaggctgctgctgactggaaagccaggggaaattagcgttctggcttcaggtcacgatcaatgtactgcctcacagcctcttggtttacntggaaaataaacctcatgtcctttatctggaaaggggnggnaaaaggtagctaaattagtanagcatgaagatacttaattaaatgcatcagtgatatctcagtcaaataacaagggaaggattgtcaggtatagcaaaggttaacttgtcaaaaagtaattgtttcatgtctgcttacanatcaccatagtatcattcgtactgtttttagatactctataaanccccaaaataacataatggcaagaagtaaancttcaagcaccctctaccagtagaaccataaactatgacaggatcacaggaatagttacaaaaactgtgcattgactaaccaccaggttacagattcattnaaaaatgaaggtatactagaacggggaagtattggtacctcgattaatgagtctgagcttaggttgatgcgtttgcagcttggtatttccttgctattaacaaagattggacattttccagtgttcttaatatgaaaata

SEQ ID NO: 36 - DNA, 774 bp, Zea mays
  misc_feature (281)..(652): n is a, c, g, or t
  misc_feature (500)..(698): y is c or t
  misc_feature (568)..(568): r is a or g
agcatcatggagtacggtcagcaggggcagcgcggccacggcgccacgggccatgtcgaccagtacggcaacccagtcggcggcgtcgagcacggcaccggcggcatgaggcacggcacgggaaccaccggcggcatgggccagctgggtgagcacggcggcgctggcatgggtggcgggcagttccagcctgcgagggaggagcacaagaccggcggcatcctgcatcgctccggcagctccagctccagctcggtaattacgactctggatacttcttnnntcttttgtgtgcgcgctgcttcgtcctatatataataatacatgnagttaggcttagtaataatcaattaatttaatccgtgggtttcgtgtttaagtcggaggacgacggcatgggcggaaggaggaagaagggaatcaaggagaagatcaaagagaagctgcccggaggccacaaggacgaccagcacgccacggcgacgaccggcggcgcctaygggcagcagggacacaccggcagcgcctacgggcagcagggacacaccggcggcgcctacgccaccgrcaccgagggcaccggcgagaagaaaggcattatggacaagatcaaggagaagctgcccggacagcactgagcggcgcctatacntggctgtgctgtgctgtgctggcgcgtcaaagccgtactcttcagygttccatagataataagataaacccatgaataagtgtccctaccctttgatcatgtgacagggacagggacaggga

SEQ ID NO: 37 - DNA, 460 bp, Zea mays
  misc_feature (53)..(449): n is a, c, g, or t
  misc_feature (375)..(386): r is a or g
aaggcaacattctgaagatgcagcgcaagcagaagccatgcactcccctcccntccaacangcagagtcggtactaccggccncgggtcaaggtangcgncagnanccgactcctngaggcnannttccccgcagnggcaagannnnnnnnnnnnnnnnnnnnnnnnnnnnntntcnnnntgnnnaagnntnnctgnnnctgnctgtctntgtgtgttcncgctttcnnnngcaggggaggtttgtcagcaaggcttgtttnctccagcgacagcaagcgttagagaaggagagctagagaangatggatcctgctccaaggcgcatttctgnggctctcttggagaagcagcagagcttctccnttttcatctrtgcggcggtaragtgcggcagatgtagagatgcctgtagagtggtgcttgtnancctcaattctcagtttcttntatccattcca

SEQ ID NO: 38 - DNA, 553 bp, Zea mays
  misc_feature (78)..(542): n is a, c, g, or t
  misc_feature (309)..(309): s is c or g
  misc_feature (342)..(342): m is a or c
cacaaaagagaaggctctcaaggtgaactagaacagaatctcccgacggccggggctcaaaccagctcatcctcggcnatatctcgaggattcctcaccagctcgagcatgctcacgacctcacccatgccaggccggttcgacggcacctganaggtgcanacaaggcccagcttgatgaccggcagggcctcgtccatggggaactcgccgcgcagncgnggntcgacgcagtcctcnggcctgccttcctccagcgcncctctgaccaggtcacacaggacaaccacgtcgtcttccaagtactcsacgggcctcctgcccgtcaanncctccagcagmagcaccccgaagccatagacgtcgcatttctcggtgatcttcaccgtcttgcacgcaaactctggcgccatgtacccgagcgcgctctggaccttactgctcaggacgtaccggtccagcatcggcagcagcttggcgaggccgtagtcaccnacctttggctcgccgttgctgtccagcagcacgttgcttgacttganattgtagtgga

SEQ ID NO: 39 - DNA, 622 bp, Zea mays
  misc_feature (4)..(619): n is a, c, g, or t
  misc_feature (445)..(445): b is c or g or t
ttcnntngcattcntngctgatgtttnngantgnctcttaggacaagtgtggctacaccggagcatgtcgaagaggcattcagactgttcaatgtntccaccgttgatgctgcaagatcnggaatcaatgagcatttgaacctgtcaccggagatcgcaaangaaatcaaggttagtatttgcatcccagggtnnncaaaatncagctnttgaaccttgnattttcctgaacggcnttcnncatttttttgcnnatctgncagcnagcggaggcncaaataaagagaagaatgggcatcggcagccacatatccnagcgacggctnatngatganctaaaccggatggggatgaatgaatccatcgtaggaaccctgtcatcgnatcttagaactgaaactatggttttcaagtaagacccgntcgtttttctgacaatatcttbcacactttgtttcaggtcagaagagcccttctgatcatgcatcaaagngacgaggtggagtacaagagagagcgccacgtgatcgtccgaaaggcttgaggtggagagnngccagtcagattcacggcatacaacgtacactggaggnggtccttccnnntcgnacgtgtgtanacc

SEQ ID NO: 40 - DNA, 664 bp, Zea mays
  misc_feature (24)..(642): n is a, c, g, or t
  misc_feature (602)..(602): w is a or t
ttcctctataagtacccgccccanatctgcgccattttctcatcgcagaaatcctccgcaacttcacagcgtatcatcgttttncatcgctcctactcctancatccagaaaatctgagnggtattgatggcgcccaaggcggagaagaagccggcggcnaagaaggtggcggaggaggagccctcggagaaggcggctccggcggagaaggcccccgcggggaagaagnccaaggcggagaagcggctnccngcgggcaagtcngcnggcaaggagggcggcgacaagaagggnaggaagaaggcgaagaagagcgtggagacctacaagatctacatcttcaaggtcctgaagcaggtgcaccccgacatcggcatctcctccaaggccatgtccatcatgaactccttcatcaacgacatcttcgagaagctcgccncggaggccgccaagctcgcccgntacaacaagaagcccaccatcacctcccgcgagatccagacctccgtccgcctcgtcctccccggcgagctcgccaagcacgccgtctcggagggtaccaaggccgtcaccaagttcacctcgtcntagccnccttgtwgtaggcgtcgttgtnnnctgcttctcaagcaagcactgtnatgtgccgcttctcatggcagt

SEQ ID NO: 41 - DNA, 722 bp, Zea mays
  misc_feature (13)..(708): n is a, c, g, or t
  misc_feature (190)..(190): r is a or g
  misc_feature (580)..(580): s is c or g
aaacaacacagtnatctgatcgtnataaaatgatatantctgtctataccgcacccaagtgtttcagtctttcagagnnccaaaacgttcgantcttttctttanccnatcttcttcctcccgacgnnncaccgccgcngnnnnnnnnncnnnnnnnnccgcgtntgagttccaacactcgagtgaggtrtannnnnnnnnnnnnnnnnnnnnnnnnnnnnannnnnnncttnccgaantgntatnnnnngtaatacatgacaaaacgacggttaattcttgtgtaacaatgcganacgagcagggcngatgtactacaacgnnatgtaccatctcttctaccagtacaacccgcacggcgcgctctggggcgtnggcaacctctcctggggccactccgtntcnggcgacctcgtnaactgggccgcnctggacacggcnctggacccgacgtcgcccttcgacgccaacggctgctggtcgggctccgccaccatnctccccggcggcaccccggccatcctctacacgggcatcgacgccaacggggagcaggtgcagnaacgtggcgttccccagsgacccggcggacccgctccttcgccggtgggacaagcccggctacaaccccgtcatcccgctccccgccgacgtcccgggcgncaagttccgggacccntcgacggcgtggctcggccgcgacgggcngtggcgcgtcgcgt

SEQ ID NO: 42 - DNA, 940 bp, Zea mays
  misc_feature (195)..(730): n is a, c, g, or t
  misc_feature (238)..(238): r is a or g
  misc_feature (266)..(268): nng is ttg or all three nucleotides are absent
  misc_feature (808)..(808): s is c or g
ctgtcatccatgtccaggaggtctgttgctgcacacccttggcatgatctggagataggtattgtacacgctctagcttgacaaatggtcagccgttgatctctgctatttgcaaccagagcttaagttcatcttggattcatgcaggtcctggtgctccaaccatattcaactgcgtaaggccaccctgtcatnngcttgactggtcctcttgtgatatgttcatgttaatagcatratgtcttttgttctattggaaaataaanngtctccctggactctaaaatcaatgcctgtgaacacatgaactgtttgtgtcacccatgttcctctgctccttggcactttctgatgcatgctcaaatgcttaagaaagactcatagaagcgactcctattcctatgccaggtcattgagataccaaggggcagcaaggttaaatatgaacttgacaagaaaactggactgatcaaggtaaagcaatgttgttttcctcccgctgaagtcttattgtgaagctatatttcttgccagttctaatatttactcctttccgtttcaatctgtgtgcatgtgcaggtggaccgtgtgctgtattcatcagttgtttaccctcacaactatggattcattcctcgcacgctttgtgaagacagtgatcctttggatgtactggttataatgcaggtatgcttcttttttatatatatcattggnngattcacaaaantggtacatcagtagtgatctgagtatccttgggcataagttgagctaattttcaaatcttgtcattttccatttctgsgaatggtcgagaacatgtctataaactgttacttccaagcatgtaggagccagtcattttccatttctgtttatagttgcctagtcgggaacatgtatgtaaactgttacttccgtgcatgcaggagcctgt

SEQ ID NO: 43 - DNA, 805 bp, Zea mays
  misc_feature (150)..(801): n is a, c, g, or t
  misc_feature (708)..(708): m is a or c
ggatccatacaaggtgcttttttttcgatttagaattctttcttcatcgattttgccctatgtgctagatcctcaaatcaattccgcatcttgtttccgcccttgattgatgcattcgctcgtctgacttgattgatgcgctcgatctgngggactcttcgttcttgcagcaccgcccgtctagtgggagcaactccagcttctggaccaccaactccggcgcccccgtctgnaacaacaactctgccctcaccgtcggacagcgaggtcagaccacaacccctctctctgtttatcctgtagctgacatgctgctgccttcatttgtcnngtctctccatcccggtttcnttttcccttgcacgatcctgtatgtactcactatgtatgnagcatatatgttcttgatttgtgcgagacccatccgaggcataaatgatctgtnctagctttgctttgaggcctattattgcaccgtggaagcnagaggatttcgnttcccatncattcaaagcttgcatctngatgtgcttttaattaatttccagtgactaattttgcctgctcngtacatgcgggttgtcgttgattnacctgtccnaatatcgtcaatgaatttgagacttgcccaaaggacttattccttgtatcagctgtaaggtgaagcttttgtcctgatatttttgccagtcgctgtcgaaccattamgttacttaagggaaagaaagcacnttccnggtacgaaatgccatcatggagtcatagtgataatcctaggtgagggacacttggagagtagtnaagt

SEQ ID NO: 44 - DNA, 860 bp, Zea mays
  misc_feature (10)..(117): n is a, c, g, or t
  misc_feature (266)..(266): m is a or c
gtacctcctnnncttagtcngctagcgagagagannnaatcctggcctcacatgagatcgactggttcctgggttccttctctcctccccccgttaagttgcccgtcggaggaggantcctgagcacatcgatcagtcgcgtgtctaggtttcctctctcaccatagcgcccgctctgtcgcccttcgttcacctctccttcctctcctccctgcctgccagggagaggggaagtcagaggcacggagtggcgcagagcagacgcmcgtgaaccattgtagctgtccctgtcgtcgtcgtcatcgtcgtcaacgaatccgcacaaggaaaagatggagaagaagccgaccatcctcatgaacaggtacgagctcgggcgcacgctcgggcagggcaccttcgccaaggtgtaccacggccggaacctcgcgtccggcgagagcgtggccatcaaggtcatcgacaaggagaaggtgatgcgcgtcggcatgatcgaccagatcaagcgcgagatctccgtcatgcgcctcgtccgccaccccaacgtcgtgcagctgcacgaggtgatggccagcaagagcaagatatacttcgccatggagtacgtccggggcggcgagctcttcgcccgcgtcgcacgcggccggctcaaggaggacgccgcgagaaggtacttccaccagctcgtcggcgccgtcgacttctgccacagccgcggcgtctaccaccgcgacctcaagcccgagaacctcctcgtcgacgagcacggcaacctcaaggtctccgacttcggcctcagcgcgctcaaggagtgccagaagcaggacggcctgctgcacaccacctgcggcacccccgcg

SEQ ID NO: 45 - DNA, 676 bp, Zea mays
  misc_feature (1)..(676): k is g or t
  misc_feature (1)..(676): m is a or c
  misc_feature (1)..(676): r is a or g
  misc_feature (1)..(676): s is c or g
  misc_feature (1)..(676): v is a or c of g
  misc_feature (1)..(676): w is a or t
  misc_feature (1)..(676): y is c or t
catctggtcctgcggcgtcatcctcttcgtgctcctcgccggctacctcccgttccacgacgccaacctggtggagatgtaccgcaagaksagmaragccgacgtcaagtacccgcagtggttctcccctgagctscggcggwtgmtgcccaagctcctcgaaccgaacccaaacaayaggrtcacratmragaagctggtckascacccytggttyawgaaggggtacasgccgsccgtcatgctggcacagccgcacggctccagcagcctcaaggatgtccaggtcgccttcagcaaygcygaccacaaggacagcagcavcaaggtggaacagccggcggacagctccttgaagccggcgagcctgaacgcgttcgacatcwtctcccactssrgagggttcgacctgtcaagcctgttcgaggtggaccaagagcagaaggccagcaactcgcggttcatgaccsaraayccggcgtcggcgatagtgtcaaagctggagcagatcgctgagacagagcgcttcatggtgaaraaacaggacgggctggtgaagctgcaggggtccaagcaagggaggaaggggcagctcgcgatcgacgccgagatcttcgaggtgacaccggcctttcacgtcgtcgaggtgaagaagtcggcaggcgacacgctggag

SEQ ID NO: 46 - DNA, 742 bp, Zea mays
  misc_feature (386)..(386): s is c or g
  misc_feature (516)..(516): n is a, c, g, or t
gcaatgtgaatgaatatatgacgcaccattatgttatgtgtgacatattttgatttctatacttctaagtattctctgatcatctgggacgtgtaaacataaaaagataataaactaactgcattcgagatcatgaccagtaataacaaacaaatgtaatctgcagtgagaacagataagtggccacataaccaaaaccttgagtctgcacagcatcttaattgtcacttaacacaagaaaacaatttagacagttataagcaacatataacattgaccattgatcatttaggttaacatggggacaagacataattgattgctaaatctatctgtaagctttattaatcttataattcataattacaatgagttcattgcaaccstcaaggtgtaatgttacagcaagtcaaccacagcagcacagaacaagaacatgttgtagacctaaggttttagtctccctttgaactctattactcagatatagagtatatatctaacaaaaatggtacnggaaaagcatacctaagaaaccacaagccacagaattgatgtagcttcgagcttcaattgaatccagacctaggacaattatgtggaactgactgtagaactctatctctttatcttcaatcctgcaaaaatgaggaactatgttcaccccattaactcgctccataaccctcttcgctgctacttcagccttggacttcccaacatcttgaactctgtacagcag

SEQ ID NO: 47 - DNA, 808 bp, Zea mays
  misc_feature (87)..(87): r is a or g
  misc_feature (182)..(762): n is a, c, g, or t
gagaagcaacatgacggcaagctcagtggctacattcgaataaggagcaagacccagggaattgcactcagcttaggggacaagatractctcaagcagaaaggtggcagttaactgtgacaagtaatcgcagttgtatcatcatttttcgcatttaggaaatccacgtgccagagagagannccagtgccgtggcattgaactgagtataaatgcttttttgtacaaaaggatcgatcaaagagagagaganntaagaggacagttatgaggaggaagtcacnnnnnnnnnnnnnnnnnnnnnnggtgttagagacccctgagcgcgaagttgtcggtcgaagatccatgttgctgtagtaacgatgctgttccaancttccttgaaatagttgtgaagtttatgttgatttctcgacaggtagttcaattgtgatcttgtactattacnnngaatccctcttgttttaatgttttatttgcctttttattttagttgtctggacttggaaacagaagcttggaggncggtgttgtcacgttatttttgtagagatgaattggagctcattttctgttacgtatagatttgccaattgtgttaggttatttttagcgtggttatttgagaaatgaggtagtccattatcttctcactcactttcttcttttgtttgtggaatgaaatgaggtaatcaaactgaancccgaaacgaagatggccttaggctgacgatgagacccantagaacttccnnnnnnctactattactctactagggcctaggaagtgatcatgatatggttg

SEQ ID NO: 48 - DNA, 1088 bp, Zea mays
  misc_feature (83)..(1064): n is a, c, g, or t
  misc_feature (472)..(472): r is a or g
atagtgcaaatctgagtgttaaccataataacacaaatctgagtgtcgcacagagaaaaggataacgcatgtagcagatcaancatatttataatcatagtgcatcgcagcccaatattgaaacagataaaaatacattaaccagtagagagttgtaccaagagagaacagaacttacttcctgagcctgagctggggtggcgactttgccagttccaatagcccagactggttcataggcaagaacaacgttgctccagtccttgatcttctctgtaaaacaaacagccatttgatccattcagcctgatttttcgtatagggtcaaaaaaaacttggtaacttcaaagcaaggcactaaatgttcacatgaacaaaacaaagggcagacccagctcccacatgaatgtggggtctttcccccacaaatgcggaaaggaaaatccagcatgtaaattcatccaagcaacaraaacaaaaactcggccggggaaggaaacaccgccctcccggtattctattaagaagagaccgaaacatggtcccggccgaaaaaatccccgaaccctagccccccatcactagttggccgtcatcgcccactctgcaaatgcccaaccggagggtggggntgcatgacataacccgagagcgggcggggcacaacgaagggattttttaaccaagcccgaaattcgccctcaagggggatcgaacccgggacctggaggtgctacttggaagctttaaccattacgctaaaggccctttcgcagcgacagaaacacacataagttgattcctaaactaaagctgttacagaaaaacagtaatgtccgaactccggatatgtagattatctaacagaactgatcaccagaagcaaagggcctgttcagtttgggtttcagctgctgtggctagctgcagctagcttataactacagtaactctactgtgacacctgagaggcagcagccaacgactgcataaatgccaaccgaacaatctcaaccaaaagatgtatagctacatttatataatgaaccaacaaggcagcaacncttcattaccattaaaaaactaac

SEQ ID NO: 49 - DNA, 935 bp, Zea mays
  misc_feature (84)..(804): n is a, c, g, or t
  misc_feature (166)..(166): s is c or g
  misc_feature (224)..(224): w is a or t
  misc_feature (650)..(892): r is a or g
atcaagagcagcagctgctttgctgagaaacaggctgaccccgcatttgcacagttgcaggcctactagcaccacttgcagctnggttgacttgccatcctatccaacaaggagaatgaagaatgattaggtgctcccgtatacagataaacaatagcaaacatastgatcatgggattcatggcttatttttcactttgaatcatatgcaatattatnnngtwgcacagtgttctttgtttgtactcagtccctcaataaaagagggcctccatatgttgacatactatacttgatgactcnnnaaggaatgagaaaatgctgccacaaaaaagtctacaacacaaatgatctagttacctgttctttatctcccctgccatggtcatgaatgccttctccacatttgttgcatccttggcactagtctcaaggaatggtattccgatgtcatcagcaagggcctatgatgacaagcaacatgcagccaatttaactatcatcccggttgaaagaagcatgtccagtaaaagtaattaatgcagagaaatattaccttgccagcctcgtaagaaactactctgttctcagccaggtcacacttgttccccaccaaaagcttgttcacattttcactggcatacctatcratttcattcagccactgcttgacattgttaaagctctcctggtcagttacatcatacacaacctatagaaatacaaaagtttaaacaagactcagattaacaaagatgagataatagcagataggaaaaaaancgaaataagaaaaagaaagcntcacaataatgccatgagctccacggtagtagctgcttgtgatggtcctaaagcgttcttggccagcagtatcccactaaatcagaaraatgtggagaaacataagtgtcaaagcttctaactgttaggaa

SEQ ID NO: 50 - DNA, 579 bp, Zea mays
  misc_feature (541)..(541): w is a or t
  misc_feature (556)..(556): n is a, c, g, or t
cgacgaggagattctcgggcttgaggtcgcggtggaagacgccgcgggcgtggcagaagccgacggcggagatgagctgctggaagtacctgcgcgcggtgtcctccttgaggcggcccttggcgacgcgcgcgaagagctccccgccgcggacgaactccatgacgaagtagatcttggacctggtggccatgacctcgaagaggcggacgatgttggggtggcgcacgcggcggaggatggcgatctcgcgcttgatgtgcgggacgaggccgttgcgcagggccttctccttgtcgagcaccttgatggcgacggtctcgccggtgtcgtcggcgtggcgggcgtggtacaccttggcgaaggtgccgtggccgagcaggcggcccagctcgtagcgccccagcaggaggcccccgcgcttggcgggccccgaggaggaggccggccgccggggctgcggtgacgcgtcccacgacggcggcggggtggcggccatcaggtagaggaggaggtcaggcgcgcggagaaacggagcggwaggcagaatggccgnttaggtggtggtggtagcgaggg

SEQ ID NO: 51 - DNA, 319 bp, Zea mays
  misc_feature (21)..(279): n is a, c, g, or t
  misc_feature (111)..(111): s is c or g
cacctcggacaccggaattcncccctgtagatcttacggtacatngccatgaggttctggtcatgaaaaggaaggtagccagccatcagcacgaacaggatgacaccacasgaccatatgtccgcctnggcgccgtcataaccgcggcgcgcgagcacctccggggcgacgtagganggcgtgccacanaaggtgtggaggaggccgtcggggtggaactgatcggccaccgccgagaggccaaaatcgganaccttgaggtcgccgcgctcgtcgacnagcagattctcgggcttgaggtcgcggtggaagacgcccc

SEQ ID NO: 52 - DNA, 614 bp, Zea mays
  misc_feature (44)..(568): n is a, c, g, or t
  misc_feature (442)..(442): s is c or g
gccaaacaagcactcttctagttcttccgtttctcactttctcnnnnnnnnnatctcccctttatatgaataatataaatgtcannnnnnnncataagtaaataaacaaataaatcaatcantattactacgaagctgtcctcaccgccttctctctccctccgaatcnaaacgcggacgcaaatgttgctccacgccggtccctcgttcctgctcgcaccacctccgcgcttngccgccgctccgtcgtcagcttcgccgaggcgatccaggacaccgcaatcctcgccgncgangtcgcatttcgcgcgccccgctgatcccgtggcccanagggngcgtcccgtcgcgcngaggccccccatggcgacggcggangagggcgccagctctgangtnggngtcgccgtcgccgagtccgcacaggttcggccgccactgsccctcctcacatnncagagtttacgcaattattatcacttgggncactcgtttgccaangattacgcgattacgcctaacctgtcggtcgggtctacatngtagtcacactcacacgaatgccccnaaccgtttgtgagctcgtggtgatgatctgtgttccacctgcacca

SEQ ID NO: 53 - DNA, 710 bp, Zea mays
  misc_feature (1)..(710): s is c or g
  misc_feature (1)..(710): y is c or t
  misc_feature (1)..(710): r is a or g
  misc_feature (1)..(710): m is a or c
  misc_feature (1)..(710): k is g or t
  misc_feature (1)..(710): c is a or c or g
  misc_feature (593)..(617): n is a, c, g, or t
agcatsaccagaagcagagcctgatggacaaggcgaaggggttcgtygyggagaagatcgcgcacatccccaagcccgaggcsacgctggacggcgtgacgttcaagggcctgagccgggagtgcatcacgctgcacagcagcgtgaacgtgtccaacccctacgaccaccgcctccccatctgcgaggtgacctacacgctccggtgcgccggcaaggaggtggcgtccggcaccatgccggaccccggctggatcgccgccagcggctccaccgcgctggagatccccgccaaggtgccctacgacttcctcgtctccctcgtcagggacgtcggccgggactgggacatcgactacgagctccaggtcggrctcaccgtcgacctccccatcgtcggcaacttcaccatcccgctctccacctcyggcgagttcaagctccccaccctcaaggacttgttctgatctagtagtagctcgcttgccttstgttctgtgcgggcgcgcaccagcgatctgtacgacgascttttgcaaataaamgamgcagctcctctgttctatatatctmagkgratgsmtrrkytaaknnnntnnntgrytnnrynnnnnnnnaaataaagagctggatttcrttcaggttcctgtctcyaagctggattycattsgggcatccaccrtgatstggatgtgcctgccgcgtccgtc

SEQ ID NO: 54 - DNA, 838 bp, Zea mays
  misc_feature (8)..(825): n is a, c, g, or t
  misc_feature (126)..(126): r is a or g
acgacganggcggcgtacnccttggggatctccgcgacgccggagaagccgaactnggcgccgatgaggctgcccacgacgatctggcacgcgagcatctgggtgccgccctgcaggaacagcttrcggcggccgaggcggtcgacggtgacgatggacacgaaggtggcgaagacgttgacgaggcccgtgatgacggcggacatgagggaggcgtcgtccgcgaagcccagcgtcttgaagaggacnggggcgtagaacatgatgacgttgatgcccgtgagctgctggaacatggggatgncgatngccatgacnagctgcgggcggtagcgcggcngcaggatgttncgccaggggtgcgccaccagcttggactcgtcgctggcggccaccaggtcnctgtactcctcctccacgtcgtcggtgccccgnacgcgcttgagcatccgcttggcggcgtcggtgtagccgcggtcgatgagggagttgggngtgtcgggcaggaanagcgcgcccacggcgatgatngccgccggcacggccgcgagcgcgaggctgacgcgccagccccagccgcccntnatcttggcggtgccgtanttgatgaggttggcgcanaggatgccgatggtgaccatgagctggaagccgatgttgagcatcccgcggaggcgcgccggcgccatctccgagaggtagacgggcacggactggttggcgaagccnacgccnacgccgaggaggacgcggccgaggatgagcatgcccacgtccttggcggcgccnttgagcgcggcgccnacnaggaacgtgacgccgccnccgaacatggacc

SEQ ID NO: 55 - DNA, 844 bp, Zea mays
  misc_feature (69)..(824): n is a, c, g, or t
  misc_feature (193)..(193): r is a or g
ccagttcaagacagaggagatgaccaacatcatgaaggacttcgacgagcccgggttcctggccccgannccggcctcttcctcggccccaccaagtacatggntcatccaaggcgagcccggcgctgtcatccgcgggaagaaggtnnnnactgatccgtcgtcgtctatgctccccctctcgatctcccartataatgcacgtcgatcatctttctcttgtttccctagggatctggaggcataactgtgaagaagacagggcaagcgatggtggtcggcatctacgacgagcccatgacccccggccagtgcaacatggtggtcgagaggctcggcgactacctcgtagagcaaggcctgtgaatggattcatttaacctcgctcgctcgcttgtccatggttcgagcatccagcagcaacgataccaacatcagcattatttaattggtagcctcctctagctacgcacgcattttnagtcccctacacgcccttggattgtgcgtggctctgttaatcatctctcatccttcgtctgccatttctcccctgcccgtcgccgatcaccagagatttttgttccttgttggtaccatgcattttggcaaataattttgtaattccacccccaaattaaagtttggttgtcgtatggtttgtaaacccagaacaatatatatannnnnntgtgtgtgattgaactgttcctgtctattctttttgtaanacgggaatatatatgtatgcattttgtgtgatgcatgccttccagggcgacgactaattaatgtgcaaccagtcctccatcnnnncatgnnnntatggtgaagggctaaaggc

SEQ ID NO: 56 - DNA, 652 bp, Zea mays
  misc_feature (1)..(652): k is g or t
  misc_feature (1)..(652): s is c or g
  misc_feature (1)..(652): y is c or t
  misc_feature (1)..(652): v is a or c or g
  misc_feature (1)..(652): m is a or c
gtggaagccgccgcggctttcttgaacaaagccgtcaagccagtgcttgtaggtgggccaaagatgagggtgtccaaagcatgcgaagccttkgcagagctggcagatgcctgcggctatcccgtcgccgtgatgccttctgcgaaggggctagtgccagagcaccactctaggttcattggcacgtactggggtgcggtgagcactccattctgtgctgagatcgtcgagtctgcvgatgcctacctatttgctggccccgtattcaacgactacagctcggttgggtactcgctgctcctcaagaaggagaaggccatcattgtccaaccagagcgggtggtggtcggscayggacccgcgtttgggtgtgttctgatgaaggatttccttcatgcccttgcaacccgtctgaagaagaacactgcygcgtatgagaactaccgtcgaatttatgtgcctyyaggcgaaccacttycatcygaacctggcgagccgttgagagtgaacgtgctmttcaagcatattcaggcaatgctgtcyggcgacacggctgtcatcgcagagactggggactcgtggtttaactgccagaagctgaagctaccggaaggctgtgggtaagctcctctttcgaatcatggttttgctg

SEQ ID NO: 57 - DNA, 659 bp, Zea mays
  misc_feature (23)..(647): n is a, c, g, or t
  misc_feature (173)..(173): k is g or t
ccaacagatgctcaggtgaaccnagtccagcagcataggcttctaaacctactattaggggaaaangaaataacttatggcgtcgaccacaaacacactgatgcacgagaagtatttctagctgttgttatctgtgaggttgatcctgcggcggcggcgggctcgacacgatktgaccataaacgaactggttccacgtgtccggcacgccggggaggcaccagtggatgcaatccgcgaacttcctcgggttcgccttctgctcgggcgtcaggagcttcccctgccgcagcgtgtgcacggaggtgtgcgcgtccttgcggatctccgacagcgcggtcacgtcgacgaagcgcaccggcaccttctccatcgacctcgtcacgcgctgggcggccgcgaagaggtcccagtccgtgcccacctccagtttcttcgtgtagttgatcgccggctgcgtctcggagaagcattttacggcgttggggctgccccagccttcactcctggaccacaacaagacagtgagtgannnnnnnnnnnctgtggaggggcagaaattctgcatatcaagcaaggtacggatggatacttactgcatatgtaccggtgacacgctcatgaataggaccgtgcttctcttgggnatcaatgtgcgc

SEQ ID NO: 58 - DNA, 600 bp, Zea mays
  misc_feature (21)..(486): m is a or c
  misc_feature (34)..(34): n is a, c, g, or t
  misc_feature (173)..(173): k is g or t
ggatctggacaatatttcacmagccaaaaagacnaaaaaaaaatcaagcacctgtcttccatccaagcaacactgtacaggtcacccaagcaagtgtcatactccggtggagggctcgggaactcgccagggcagtatgtcccccagctgctctcctctgcatttgacgcggkggtcgcatacacattgatgtcattcggcaggaggccctcaaagatgctcccagattcgcatgcttcaaggtaaaagacctacaaaaggtgaaagaatacacatatacctcaagcccttgctttacatatcacaacatttcagagcagaactgaacaaacagctaacggtaccaggcttttgtaggtcccggcagcatgcttcttcttcaggacatctacgaggtcatcaccatagagatatggatacgtaggcattcctgaatttttttacagagtaaataactgtgtctattttggttctacatgcatgtamgaactgatattttatctaagaaacatctaatctgaatgaaatcagtagcaattagttgcgagtacagaccaaggacaccaggacccccatggtcactgtagaaaacaaagatat

SEQ ID NO: 59 - DNA, 890 bp, Zea mays
  misc_feature (1)..(890): k is g or t
  misc_feature (1)..(890): m is a or c
  misc_feature (1)..(890): r is a or g
  misc_feature (1)..(890): s is c or g
  misc_feature (1)..(890): w is a or t
  misc_feature (1)..(890): y is c or t
taactgctaawaactataggcgggattatcatctgggttcaaatatttggacttatgtgctcctttgaggcggcgaggcagccacacccacacgcagtggcctgtggcgcctgggcggtgagtccgcctatgactgcgaaygttayrattttattrggcatcctttttagttgattgrattggttgtagcytgaaccttatctaccattytatctcccctgcttgtsgtgttytatgtccctgttcrgcagctcatcccagcgctgcttggcagccataccayagtscttttatgctcacagaggcagcagcagcagcagccgagacakyagtggcttgaagtgcagccragaygrmytattggcattttatctrtctctyctgagakatgaaatgrgacattgtaggtttatgcatattcagccrcctttgctagttattatgtgattttgtaaayttcctgagcctgcsactaaattatttcaacatatttagtaatgcgmtgggagtatatgcagaasttaagtaccttttctgtttgttttgtcaacaaagtgagcaaaaaaacaatgcttygttwtgtgtggccatgttgcatgagtgawgaagcacrtgtttctttcttttcacctgaaaagtaaaatarttctgcaagyagaatctckagttayggaatgttatttctgaatmygcagttcrcatcatgttcagtcaagtactagcactgarggttgcttcctttttgatatgtgcagaaagcacttgcaggtctgagaagaatcaatttagatgggcttcgatggcgcgtatttgatgctaagggtcaggttaggattgtttttctagyttgartagcatggatgaacttatctcaagaaggatagaggcta

SEQ ID NO: 60 - DNA, 505 bp, Zea mays
  misc_feature (267)..(505): r is a or g
  misc_feature (387)..(411): n is a, c, g, or t
  misc_feature (481)..(505): k is g or t
  misc_feature (481)..(505): s is c or g
  misc_feature (481)..(505): w is a or t
  misc_feature (481)..(505): y is c or t
atcaacgtgcagaacaagaactcgtcctacttcgtggagtggatccccaacaacgtgaagtccagcgtgtgtgacatcccgccgaggggcctgtccatggcgtccaccttcgtcggcaactcaacttccatccaggagatgttccggagggtgagcgagcagttcactgccatgttcaggaggaaggctttcttgcactggtacacgggcgagggcatggacgagatggagttcaccgaggccgagagcaatatgaatgacctcgtrtcggagtaccagcagtaccaggatgcgactgctgatgacgatgaggaggccgagtatgaggacgaggaggagccagctgatggcatgtgaggggaggctgttaaatgtgaagcctggtgnnnnnnnnnnnnnnnnnnnnnnnnnatgtcccctttcgtgttgtcgccatgttatactagtacactagcataccaccctcgtggcccattccgtcgatsgtrsytgttktrsctkgwgw

SEQ ID NO: 61 - DNA, 547 bp, Zea mays
tagggtcctgctacaagagatcgccacattttattgctacggaagtccagttgtgtctgtctgtttggtggtcatggatatggttcggtttttactgctgtaaaaagggactggggaaaaaatgcaaactgacttggattttttgttctgttctgcatgaagatgaaatggtagggtcgtcggaggaggacgaagcatgctcgggaggagacacggaggcgacggagccggggcagcaggagcacagctcccgcctggcggaccgtgagctgaaggagatgctgctgaagaagtacagcgggtgcctgagccggctgcggtccgagttcctgaagaagaggaagaaagggaagctgcccaaggacgcgcggtcggcgctcatggactggtggaacacgcactaccgctggccgtaccctacggtaaccatgcatgcatcctggcaaacacgcagcagcagcatcgctcgctggaatggcagatctgtgaccagcattagccggcggtgcaggaggaggacaaggtgaggctggcggcggcgactggg

SEQ ID NO: 62 - DNA, 490 bp, Zea mays
tagccgtcctgcaaacctcctggataaagtttggaccttatttaggaagagaagcaccctggacgagccgcgtggtatcaattcttgccgctctcctccgctttcatcttcttctcccacctacgtttctggtggaaaaaaagtttcaaagcacgaacagagagatgagccagttagatcttttttcaagggatgccttcgttcaatcactattacagctatcgttacatttgatctgaaaacacaaacatggcatctttgtgcaccaaggtcaatgcaggataaaaagctggatcgctgacaacagatatttgattgtccgttggaaaatattttttcaatggccacagttttagaaaatattttcccaaaattatgtcattactattactagactagcaaagtagataatggcgagcaaccatcaggaaatcttgccatcagtgcagcagaactgcagacccttatattagcgcaccagcagaatcta

SEQ ID NO: 63 - DNA, 420 bp, Zea mays
cgagtggtttgaggttggcacacaagtattgaatattgataaatcacacatacatctacagggcggacaaaggtgacaccattaaagtgtcaggtgtttatcaccttgatgagaaacagaaggcctcagctgtggctgagctaacccggaggctctcaacaaatcagaacacactcacagtcggtggactgtacacagttgatccccagacagctgtgaaggcaagactcaataacactggaacgcttgccgcgcttcttcagcatgagcttaaacccaagtcgctcttgacaatctctggtgaattcgacacaaaggccctggacagatccccaaagtttgggttggcgcttgcactgaagccctgatcagatcatcccatgttgattggtggtgaatcttgaattcattttttttttt

SEQ ID NO: 64 - DNA, 1015 bp, Zea mays
cttaatatgtgagttttctaagttagcaatcttatatatttaggcactgtatgcgactgttgtttgacaacccttaagcttatttgatacctgtaatatctttattgatggttaattgcaaatccctgcttgatgcatctcaacttcaagttgttttgtagctggtttagtgcataaaattagtcaaaatattaatataccggtcaccgtcatttcaccttttctcactgacatttctcaaatggagttttgaaagaaggttttacttcacttatatacgtttgcaacaaacatgagtttctaactcactcagattataaaaaaactcagccggggagggaatgaccgtcttgctggtattatattaagaagagaccgaaacaatggtcctgccgagaaaatcctcgaaccctggcccccatcactaacggaccggtgtcaaccgtcaactctgcaacggcccaaccggagggtggcgcataggacatcgtaacccgagaccgagagcggatggggcacaacgagggaatttttttaaccaagccgaaaaattcgcccctgaggtgttactcggaagcctttaatcactaggttagaggccctttcgcaactcactcagattattgcatgtacagaaattggtcaatgtaactgactttgctagtgtttttagtttcactgaaaaaaggatctcttgcagtaagctggtagcagtatggctaatattaagctgtgcctccagtaagggtttggtgctcagcattttgtttttctaattgagtcaaaagtcttatgtataatcttatattaaatgaaattgatgtcatagttcctcaacagatataatcccatttttaaggacgtttaacgtcttattattgcagttacatccaaattttctgtaacttatccaaccttctcttgcaggaacaacaagggagacaaccttactggagcttactaccacaaggtgagcgaattgacaaacacagctgttggggcagagcttacccac

SEQ ID NO: 65 - DNA, 900 bp, Zea mays
acaactacaaggacctcgaagccgaggctgctgcggcgacggaccaggtgccgccgtccatcgtcaaccccctgctcaggacggggtaccacttccagccccccaagaactggatcaatggtaatgtaaagctactaactaatccaccacccaacgtcgtttgaaggtgatgtgtgtgttaagcatctcctgaaatatataagagagcgaggctagtaatcggcttgttgttcagggttttggtttaccacttgtagcctcaactaataaagctatatatatgagagcgacgagagagaagagacaaaacattcatgagtatggtcagacagactagctagctagacacggcagagaaattacgagagttaaaaaaaatgcgcttgaagggtgaaccaaaacaaaacaactttagtactatgcgtcaacaaagctgtgttcatgtgtcagctagcactagagtcatagtgcgtggccagtgagctgttgtctagcaaccaacgcgaactgaagtttgagagcgtactcgtgttctcgatctcttgcagcgcaaaggtcttcgtacgtgatcaggaatattgcaccatttactgcttaattaattaagtacgtacgtactgtacgtttggctctacctcatcttctaatcttttcggtgctgtcttgtgctctctcggctctgattgcatcgatcggcggcggcgtgaactttgcaacggcggcagatcccaacggtaataagtcgttttccccaccctttttatttcctctaataatgcatcaatattccaactgggtgcatatgcatgcgcgcagcgcccatgtactacaaggggtggtaccatttcttctaccaatacaatcccaagggcgccgtatggggcaacatcgtgtgggcgc

SEQ ID NO: 66 - DNA, 344 bp, Zea mays
gggcaggcgtgtacaagccgccatacggaggattcgtggacgtcgacgttgaggagcacgagaccatcaatttgagaaccctggtgagtttttttttctttttacttttttgctgctttgtccttcagcgatctgctcagttcgtttgtgatttgcacagattgatcactcggtggtggagagcttcggagctgacgggcggatgtgcatcacggctagagtgtaccctgagcacgcggagacgagcaacaaccacatgttcgtgttcaacaatggcacaggcacggtggaggtgtacaagctcgaggcatgggagctcgcggcggcgaccgtaaattccgttg

SEQ ID NO: 67 - DNA, 7375 bp, Zea mays
aatgtcaagtatatccatttaaatatcattaggtcccgtttgtttcctttcattttaaggaattggaatcttactaataaaataagctatttttttagaatacgagattccaccactttccaaagttatcagataagcctatctcaaattcatggggtgagagatggaaattgattctatagatttacatgttattttcccgatgtacaacttatatcatactctcctaattgcttcgctataacataaatgcactatataactatctctcttatatgatttaggataatatacaaatatattacatatataaatatattaacttaattagttttgtctaaattataattattaaaatggaattcaattccaacgaaacaaacgggcccttacaaaatttctagtatcatttaaccatctattcaacacaccaaagataattggataaaatagcaacactaggacaaatactacatagcacattacatgttccattatatggtcattaaattgtcgttaagccttctataacattatggcctaaaaggttgttaaatagtaaaaaaagatggatgactaaagtccaagttcatgcttgggctaagtttatattgggtattttataccacgggttaacgggtatgggtgaaggcggaacgttctgattcccgtttacttattgggtgaagatttttgcctaataatagacctacgggtgaatatttatcccacatatatatcctagtggagtcaatatccatcggatatcggtcgtgggtacccattgccatctctagatcgaagagtagaaatttacttcctaaacctctctctgtctcatgcagcacaatagacgctttgtttcgttgcaacagcttgtttctctttgacgtccaaattcgtctatctacggacccacggccgcccagattttgaaatttcaaaacggaacacaccccggggttcggagtatctgctgcccctgcggtcctggaaagcccggcccacctctcacttgcaccaccagctcaccggttccggtcaacagtctctcgcgggtgcctgtgccggtggtcctccgtcctggctctggctgccacccacctcccgattaccgttctcgcctcgacttcaaaacaagagcccagatctaaaccaagcacgcccatctttgccacaccacacccccagtattcgaatctctcgtgcccagatgcggcaaattaaaaacaacggacagacgcggaacccctccggccaacggatctcaccctctgcggcatgggtcccactcacgctcgggtccactcgacagcgtgtagggcagagaggcgagcggtaccagtaccataggcctcccgacgcagtccgggcagcgggccccgcggattggaccggtcaaaaggcgtggcccaaccaaaccccaagggatccggcgctttgtctgcacgtgaatggtgccaagatcgcctggttgacaggtgggacccgtgaggttgtagacccacatgtctgtggcgttaaaggaggggggagggatcggcgggcgggtggtgcgcgcgggcaggcgggcgtcgcgtggtggtggtggtggtgggtgctttgactgcaggcctcggcagcaggcagagaggactagaggagtcggggcctcggaggaggggagggagagggcgaagagtagggggaaccaaatcttgaagggtaaacggagagttctttcgtggaggaggaagggggggacagcaggaggagggtagaggtatgtgcgcacccatctgttcttgctcctgatttggctgtttgttttttctgtctgttcttcgctgttggtagtttgtgaccgtgaatgggcgttcctggtccatgttcgcgtgcgctgctgccgattctgggagctctctggtcgtccgtctcgctgggatctgccttttccccggtgagagccgcggaacgttcgccgccttttcttactcgcgggccagttatggtttctggagcgttttctctgttcttggcgaggtggtcatcgctctgagaacgatgcgctctttctccgagtttgtgctcaagttttcgtcagcctagaggctatagcgtttgctgcggatctcacgacttctctcttcctcttctctattggtgcatacgttttcatccgaaatccattagttagtgcccgagccgtcaattctttgtggatttgcttgttccccttcgttacaggctcggaaatgcccctgaacagattcacaggggtcctagattaggattattttctatgactttccaagagtcaggagcacgattgctttctctcggctgtctgcctggttcatgactcagccgggtttgcaagcctaggaagaacttgctcacgtttcttacatttatctagattcgagggacgggttgtactcgttaacaaagttcacctcgttagtcattaaagctccgctgttgtgaatgatgctgccattgcgatatctggaatcatcgctctgatcgatttggttgttaatccacttacaggtagctcaatagatctactgctctcgggggagttaatgcaaagctgagttgctgcacgttggctttcttcagagatggcttcagctggtgtagccccatctgggtacaaaaacagcagcagcactagcattggtgccgagaagttgcaagatcagatgaacgagctaaagattagagatgataaggtgaagatgccttgatatcttgtttcgggcttactgtaatttcctcaagattatgtgaaaaatgggactgtgatgtaacctttggtgtgaatgccaaatgcaggaagttgaagcaaccataattaatgggaaagggactgaaactgggcacataattgtcaccactactggtggcaagaatggtcaaccaaaacaggtgagtgctttactgcatttgatcatgatttatcaactattctacatgtttttagtgcatgtctgaatctaataattgagagtcaagaccataatttaatgtccttcttttgcatattgccaatatatccatgttgctaacttataagattgtggagttgttctgatcagttttgtcagattctttttgtataataatgtgtatttattggttgcatttgcagacagtgagctacatggctgagcgcattgtaggtcaaggttcttttgggatcgtcttccaggttatttgcaataacttgtgactgactttgatatgtactattatgtagccgcctgtggtgttgctttccacggcgctgcacatgttttagatcttcatatcttgcgtgctataaatcacctttcttaatcagatgccatttcacctgttcataggctaagtgtttggagacgggtgagactgttgccataaagaaggttcttcaggataagcgttacaagaaccgcgagttgcagaccatgcgccttcttgaccaccctaatgttgttgctttgaagcattgcttcttttcaactaccgagaaggatgagctttatctgaacttggtccttgagtatgtgccggagacagttcatcgagttgtgaagcatcacaacaagatgaaccaacgcatgccacttatttatgtgaagctgtatatgtaccaggtaatggtttgtcctgttcctttttgctgttgttttaattataccttaaagcttatgttttgggccctgtttgatgttgaaactaacaaacatatttcatttcgcctaaatattgtctgctccaatgaatgtgctagttctttttcaatatttgatattatattggattttggcagatatgtagggcattggcttacattcatggcactattggtgtctgccacagagatattaagccacaaaaccttctggtatgctggaaaatctgctattttgctactgtatctttttgtaaagaaatgatttgtactttgaaattgatgttcaaacttcactacaggtgaacccacacacccaccagcttaaactatgtgactttggcagtgcaaaagttctggtcaagggggaaccaaacatatcgtacatctgctcccgatactatagggctccagagctcatatttggtgccactgagtataccacagcgattgacatttggtctgctggatgtgttcttgctgagcttatgctagggcaggtaaggtgtctcaaatttttattgccattttaaaaaaggttttcaagccaacaaggtcctttcagttcacactgtcttacaagaactatttggacagcctttgtttccgggtgaaagtggtgtggaccaacttgttgaaatcatcaaggtaattgtcggttctacaagcttgtgaattgtcttctatagaagcataaaatctgatcacccctaaaatgattttgtatggcaggtcctcggtacgccaacaagggaagaaattaaatgcatgaacccaaattacacagagtttaagttcccacaaatcaaagcacacccatggcacaaggtgctcaaatctttctacattttgttacaatactctaagaaaactgttactgttgtgttactaatttactttttgtacattttatctttcaggtattccacaaaaggatgccgccagaagctgttgatctggtctctcggctactccagtactccccaaatctgagatgcactgctgtaagtgcatgccattgtacattatacatgatggaaatacccctgttgactttggttttctaagatcttcatgaatgttttgtccagatggaggcacttgttcacccattctttgatgagcttcgagatcctaatactcgccttccaaatggtcgctttttgccaccactattcaatttcaagcctcacggtatgtttcatgcctacataattcaacatcgttatcatagctgctacaaccaggtagcagtgtagtactaagtttgttctttgtatatcaccaccttacatgctcgccacctctgttctgcagaacttaaaggagtcccatcagacattgtcgcgaaattgattccagaacatgcaaagaagcaatgctcctatgttggattgtgaaatgaccgcgccttgagactggaacctgtggttgcaattgtgaatttcccctgggatgtttgacgatctgaggcatgcgagcctgttgttgaagatgcaaggttacgtacttgtacgacaatgtgacctgtgtagctgagtagtctatgtcgcagtgacatgtaacggcaccccccttcctactaactgacgcttactcgagattgccatagttgatcttgtaatttgttatagagcagtatgaatgtatttatggtagcttgaatctatgtatggattcacttcgtttttccatgtttccttgtctccagacccagattgctaccgtattgtttcagaattcctagctacctgttgcctattgagtattgactaccagcttgcacttgtctgttattgcactggctgtggaatcagctgttgatttttgccacaatattttagttcagatgtactccctattctaaaaagaatgtgaaatcttactaatagaatagactactttttttagaatttctttccattttgaggaattaaaatcttactaatagaatagactacttttttttagaatgtgacattacaccactttctaaagttatcatataagcctatctcatttatggggtgagagatgaaaattgattatatagatttacatactgtttttccgatgtacaatttatagcacacccttctacttgcttcgctataacataaatgtagtatataactatctctttcatgtgatttaagataatatataaatatattacatatataaatatatgaacttaattagttttatctaaattataactattaaaataaaattcaatttcaacgaaacaaacggggccttgattaattataaaatgtatttttgtaataagttgatttaaagctataatgtaaatactatttactagaaacttggttaaatatgaattagtttaactaacgagtttaattggcataccacttatagttatattctttgagacggagggacgagtacgttgttcgatcggtctggaagtatgctgacttgatcgttcttaccagaaagttgcattattgcagcgtttgagacgactgacgaggaaatgtgacacgcagatgctactcagtgcttggcaggactgcattccaagtggtccttctggggagagaggaatcatagactgtagctccggtttcttgaaaaaaaacggttcccgtgaaatggcaggtatggttctccggttcctttgaaaactactctttgtaaaatgaagtatgcttggctctatcgaagttagctgttgttaacagccataccagacaggttctttcagtgtccggttagattttgaggcgtcgagggttgtttggttgagaagtggagagttcctttagagtgtgtttagttgagaagtggaggaaaatggatcgactatattcctattttttttatgtttagtttccaagaaaagcggagcagagcggctcctgaagttttagaaatttaccataaatagtttaaatgctcccgctccgtcaaaacgaacatacacgagcgctctcctccctctacttccttctacaaccgtatgtctttccaatcaagcaaagaacggagtagctctgctctattctactcttaaccaaacaaaaaaatgaagtgactctgttctgcttgtcaaatgcgaaatagaatgattctattctaaaaaattggaatagagccgctccaaccaaactaacctcactcgagggactaaagtttagtctttactctatttgattccaaggactaaaagtattcataacatattaaatgacttgaaaactaaaatgttcttaacattcttccgccattagcataactaaaataaactagggataagtgaaattaatatggactaaaacaatttggtcgctgttttattcccatatttgacaatttagaaattaaataaaactaaaatagatggattaatttttagttcctcaaacaattttttctaacaattttcgatggactaagtttagtcatttttcataagaaattaatatggactaagggcctgtttgtttacccctcagattatataatctggattaaataatcctaagaggcaaacaaacagtctagcttatttgtcgagattatataatctaactcctggattatgataatccataagcaagtgaggaggtgcttatttcagattatttttttccacttctccactaccctttcaagtttcctagaaattacccaccattgccattataacccaccattggcattcttgtcttcctcatacaa

SEQ ID NO: 68 - DNA, 568 bp, Zea mays
ggtgggaaaactgaaaaagacaatcatgaaggtgtaaattctttactatctgaggagttggaaaaactagctaatgggaatagcaaggtatgatataccctccatgattctgctttcatttattctttgttcatatggtatggttatttaacagtgctatgtattgccgtaaatgcagattcctggtacattagatgagtatagaaagcttgtcgttccaataattgaggagtattttagtacaggagatgtggaattggcagcttctgagctgaagtgtcttggatctgatcagtttcatcattactttgtgaagaagcttatatctatggcaatggatcgccatgacaaagaaaaagaaatggcatcgattctgttatcatctttgtatgctgatctactgagctcctacaggatcagtgaaggttttatgatgcttctggagtctacagaagatctaactgttgatataccggatgctactgatgtattggcagtttttattgcacgggctattgttgatgaaattttgcctcctgttttcctcactcgagctagggcactactt

SEQ ID NO: 69 - DNA, 477 bp, Zea mays
catatcccacgtttgctggctgaattgtctggccttgagaagttacttgctgcaactggcccagttccagacccatggcatcatttgcagaccctgtcagcatgttaggtggtaagaacgaaaatgtgtcatcatatggtgcctggacattggcggatgaactctgcagctgagatggatgtgttgcgctttggtcgacgccataccctgcagaatcagttccacctgaaaaaaaattatagagagcactgcattcaaatttcaaaggctcactatactgaagtagcatatttacatatcttaaagcctttgtatcaaactaaatatccatatcaatgtacttacaacaacaattagggtttccagttaacataagctacaaactgaaacgatcaagataatagagctctgttaattgtatctgagcctcagatgctgctcacctgatggtgatggccctggcatgctcatcgaaga

SEQ ID NO: 70 - DNA, 1216 bp, Zea mays
ggcgaggcagggtgtcgtcgcttccatgcatgcgctggcattgcttctcggagcattcgcagccattcctacaggtagactatacctatacgtgcatgcgcatccacccataatccgtgcatgcatgcatgattattgacactaatgtccttattactaaacaggagtccaatccatcggcgtgtgctacggcgtgaacggcgacaacctgcccccggcgagcgacgtggtgcagctgtaccagtccaacggcatcaacctgatgcgcatctacttcccggacgccaacgcgctgaacgcgctgagcggcaccagcatcgggctcatcatggacgtgcccaacacggacctcgcctcgctggcctccgacccgagcgcggcggccgcctgggtgcagagcaacgtgcaggcgttcccgtcggtcagcttccgctacatcgccgtgggcaacgaggcctccggcggggacaccggcagcatccttcccgccatgaagaacctcaacgcggcgctggccaacgccggcctgggcggcagcatcaaggtgtccacggcggtgcagagcgacgtcacccagggcttcccgccgtcgcagggcaccttctcgcagggctacatggcgcccatcgcgcagtacctgcagagcaccggcgccccgctgctgtgcaacgtctacccctacttctcctacatcggcaacccggcccagatcgacctcagctacgcgctcttcacctcgccgggcaccgtcgtgcaggacggcagcaacgcgtaccagaacctcttcgacgcgctcgtcgacaccttcgtctccgcgctccagaacgccggcgccggcaacgtcccagtcgtcgtgtccgagagcggctggccgtccgccgggggcgacgccgccaccgcggccaacgcgcagacctacaaccagaacctcatcaaccacgtcggccagggcacgcccaagcgccctggccccatcgagacctacatcttcgccatgttcaacgaggaccagaagacgggagccgagtcggagaggcacttcggcctcttcaacccggacaaatcgccggcgtaccccatcaatttctcctaattcctaaacaagacgccgaggtccattccaagacatttataaggcaatacacacacatagatatatacatacacatacatacgggagaaagtagaataaataaactgcctgcagtagaatgca

SEQ ID NO: 71 - DNA, 522 bp, Zea mays
aaggactttggaggagatactctatgctctggttgttcagaagttcgttgaagctggtgtctctctggttccagcactctcacgctccaccgatccttctggaagagttgatcagtgggcagaaactgtggaagaaaagcttcaacgtctgcactcgcatgaggcctatgaaatgatcgagaatcacctcaccctcattctggggcagcgtcaaggtgacgccactatcgcagccataagtaagctccgtgttggccaggtctatgctgcatctgtgatgtacggttatttcctgaagagagttgaccagaggttccagctcgagaagacaatgaagggcctcccttgggggtcagaagaggaagacagcgctttgaatcaagttatgatgaccgacttgatgccttcagctcagacttctagctctcatccagagatgggctcgtggaccgcgcctgccttcagcacaggagggcccagccaatctatcaagccttgccgccttaggtcgtatgtcatgtc

SEQ ID NO: 72 - DNA, 439 bp, Zea mays
gtagtccttgagcgaccagaagctgatcagcgcggtggccgccatggcgacgcagaccatgaagttgctcgtcacccacaccaccctcggcccgaccttccggcacatgggctcgatcaggaacgagctgaatcctagaacgatctgcacgtacggttcaccagcctcgtggtcagctatctatctatctgtcactgacatagtgcagcgcctggcaatggacgaaacgaggctactgaatctcaccgagttgagcagcagcccgaacgagccaactctgacgccttcgtcgaacgccgagatctgagcgttgctacccttggggtcgccgtggtagatctcacggcccatccagtcggtgtcgtagaggatgaacgggaaccaagagagctgcatggacgacacagtgcatggcagcagcgtcagccgtcagtaaaga

SEQ ID NO: 73 - DNA, 369 bp, Zea mays
gggtgcacagattgggatatgacaaatgttgtgattttcaggccaagaccaccaagaaaatcgtattgaagctgcagtgccagagctgcaagcactactcacagcacgcaattaaggtgcagtgtctcattttcctgtgttaggcttgctgttgcacaaagtattgtctcactttgatttagctcactctttcctgactgactcacctgtgtcacagaggtgcaagcattttgagattggtggagacaagaagggcaagggaacatctctcttctaagtttctcatcgcccatctcgatgttggatcgaacctgtgggtctactactgttctaaaaactcgtcaaatttcaatgttactagtagttctg

SEQ ID NO: 74 - DNA, 836 bp, Zea mays
gagaagacctgctccttctttgtcgggatggtggtgttcctggggatgagcacagtcatgacgcctccggccgtctccaggccgagcgagagcggcgagacgtcgagcaggagcagatcctgaaccttctcgttgccctcgccagtgaggatggcggcctggacggccgcgccgtacgcgacagcctcgtctgggttgatgctcttgcacagctccttgccgttgaagaagtcctggagcagctgctgcacgcgggggatgcgagtggagccgcccacgagaacgacgtcgtgcacgctgctcttgtccatcttggcgtcgcggaggcacttctccacgggctccatgcacttgcggaagaggtccatgttgagctcctcgaaccgggcacgggtgatggtcgtgtagaagtcgatgccctcatagagcgagtcgatctcgatggtggtttgggcggtggaggagagcgtcctcttagccctctcgcaggcggtcctcagccgccggagcgccctggggttgccagtgatgtccttcttgttcttcctcttgaactcctggacgaagtggttcacgagccggttgtcgaagtcctcgcctcccaggtgggtatcgccggcggtggccttgacctcaaagatgccctcctcgatggtgaggagcgagacgtcaaaggtaccgccgccgaggtcgaagatgaggacgttcttctcgccgtcgctgctcgacttcttgtcgagcccgtatgcgatggccgcggcggtgggctcgttgatgatgcgcatgacgttgaggccggagatgacgccggcgtccttggtggcctggcgctggga

SEQ ID NO: 75 - DNA, 1019 bp, Zea mays
tatagtacgttttattcgacaagcagcctctgcatgcaataatagtacaccccccgatttaattggactaatgcatgctgaggatggatcagatggagatgctgctggggatgcccctcccggtgactcccggcttggagaagggcttgagcagctcgtacggcacgatcccggcgccgcagcggttcttgaggtccaggttgttgttgcactcgtcgatgaacccctcgatctccttcatcctgccgccgaacttctcgaacgccgccttcaccatgggctccgccagccacgacggctccgcgaactcccccatgtactcctcgtcgggcgagtgcgacgagaggatgtccagcgtcgtcatgaccttgatggcctgcatctgcgtgggcagcatgtccagcagcgtcgtctccggctgcttgaggaacttctccatctcctcgcccggcccgccctcctccaccggcatgttcttccggatggtggtcggccggttggggaagtagccggcgaagtggtactggccgaagttgacggccgagtggtggccggaggtgacccacatgatggtggtcagcgtctccaccaggctgtcgcgggtgtccagcacgggccaccacggctcgtccttcttgtcgccgtgccccacgttgcgcacctcgtcccagaacgccctcagctcggggtcggcggccacggcctcgtcggacttgtagtagacgttgacgtactcggacgcccactgcctgatggagtcccagaccaggagcccgtcgtgggcgtaggggtagtccttgatggtgagctccagctccccgtcctccccgcgcacggccagcccgcgcttgatgaggtcgttgggcagcgcctccgtgtcgaactgccacgtcgcgccgtacgccacggagctgagctcgacggcgtacttgcccggccagaaggactcctcgatgatgccgtcggcgttgatgagcgcctccctggccagcgcgttgatctccatggtgtagcggaag

SEQ ID NO: 76 - DNA, 499 bp, Zea mays
gacaagctcgccatactgggtctcccgatctggattactgagttggatgtcacagcagagaacgagcacatacgagctgatgatctagaggtgttcctccgggaagcatttgcacatcctgctgtggggggaatcatcctctggggattctgggagatgtttatgtttcgagagcacgcccatctggtcgatgctgatgggacaatcaacgaggctggcaggaggtaccttgctctcaaacaagagtggctgacccgtatgaacggcagtgtcgatcaccaaggagagtttaagttcagaggataccatggttcgtacacagtggaagtgaacacgccttcaggcaaggtagctagatcgtttgttgttgacaaggatagcccggttcaggtgatcgctctgaatgtttaatgtgtgggaaatcatgcgcgtgtcctgtattttagcgatgtactgaggtgttgaacacagatagtttcatagctgatgccacgccttc

SEQ ID NO: 77 - DNA, 886 bp, Zea mays
gtcagtagttcatccatttgtcccattttttcagctaggaagtttggttacactggccttggtctaataactgagtagtcattttattacgttgtttcgacaagtcagtagctcatccatctgtcccatttttttcagctaggaagtttggttacactggacttggtctaataactgagtagtcattttattacgttgtttcgacaagtcattagctcatccatctgtcccatttttcagctaggaagttcggttgcactgaatttgtgaacccaaaagaccacaacaagccagtgcaggaggtctgtctctttacccaagacaacaaaaggttatcacagcttatgctgaacttggccataacattcaataattcctttatggtctaggtacttgctgagatgaccaacggaggggtcgaccgcagtgtggaatgcactggcaacattaatgctatgatccaagctttcgaatgtgttcatgatgtaagtatatgtatacactctcagctactttccttctccaggttcccttcatccagacatgcatgttctaactgccgcgctcgtgatccagggctggggtgttgctgtgctggtgggtgtgccacataaggacgctgagttcaagacccacccgatgaacttcctgaacgaaaggaccctgaaggggaccttctttggcaactataagccacgcactgatctgccaaatgtggtggagctgtacatgaaaaaggtaaattgcaaagtgccgttccttcagtttccttacctgccgagcttttgctgaaaaactgttaagaatcgttcctgcaattctgcttggctctgcacaggagctggaggtggagaagttcatcacgcacagcgtcccgttcgccgag

SEQ ID NO: 78 - DNA, 847 bp, Zea mays
atgcgcccttgggtacatagcaggagactggaaaggtaacaaatggaatacggacacgtagataaccatggaggcccagcaatgttgaggtattgtttggtcactgcatagccgatgatgatcaccacgcctcgtggatgcctcatgtcttaacagcagccagatgatctctgagcccggttgccacctaccacatccacggtatctggcacataccttcaagaacaaatcgataaggtcaaaaaaggggacggcttttacacagataataaaggaccagcacagggaaacaaatgaaggaaatcaaaagtgattgatgattttacatagatataatactgaaaacgagatcagcagaagaagctagtcttattgcagcagctaatgatgccaaccctggtacacccccagaaagaggatcaacagaaagtgccttattttgctgatgactaataactggagcaaaaagaccaacagaaggaccagttgatattaaaaatgtaattacttttacagcagtgctccggttttctagtacttgcaacgattaatgtcacataaaaacagtactgtcaaatgccaatcaaacaaacaaagaaacgagaataagtgtgcttacaattcttcctccggttcattcttcagagcattctttacaatacactggaaggcatcttccacgttcgttccatccttagcagacgtctcaaagtacgggatgttccctttagaggcgcaccatgcctttgcctttttctccgacacctaaaaccaaagcagattatgtttctaagcagctcatgatccagttcaagagaagaatttattcagagagcaaatcatgtag

SEQ ID NO: 79 - DNA, 815 bp, Zea mays
ggtttgtctgtttcatgaataatgttctgttgcgtcaaattaatagcaagtttctgatatttttttttctccagcatgtttttgaatactttacagaaagaaccccaagatcccatttcgaacatcgtgaaacatcatttgtgtggaactataagtatgctggtaagtgtttatcttccaaacattctttttaagcaaggtctgtgcagtaacattttatttccaccttctatctcaaagatgttgagttcggaaggctacaagcaagagatatgctgcagcacttgtggacaggtccgatctcaaatgcagctgttgatgttgttcaagggagtcgatcagttgaagttcggtctgttggagttaccaaggtaagtggtgctgtatgatggtccatgacagtagatggtttgacctagttgaggttttaaacatcatttgtctccttcctatagggtgctgcaattgatcgtattttaggggagatagttcacagcgaaaacatgattactccaattgactatgtcctgtgcatagggcatttccttgggaaggtaatttccaattcttcacgttattgttctgatctggttttagttctgtggataggatcaagaaacttatgaatgaagaaatgaaagggtttagaacattcaaaatgcattgccaaggaaaggagaaggatgtggacttaattagaaaaatcactatggtttactttatatgtttggtctgtccctattcttttcgactttggtctgttttgtaacatctggttcctcgtgtttcaggatgaggacatctacgtcttcttt

SEQ ID NO: 80 - DNA, 426 bp, Zea mays
tcttcagtctccaccctgattcaacaacagactctgacagcttgcacggtagctgccccgccatcgaaggccagaagtggtccgcgactaaatggatccatgtgaggtcatttgacctcaccgtcaagcagccgggtccctctgatggatgtgaggacgacaatgtcctctgcccccagtgggcggccgtgggcgagtgcgccaagaaccctaactacatggtggggaccaaggaagcacctggcttctgccggaagagctgcaaagtatgcgcagagtaaggtatcggtcctctgcgtctgatgagtaatcgtggcgtacgtgttacgtagttgctgtcaccattttaccagggtttaggtacgaccgagtacagcatgtataagacagtacaaacccggaagaaggaatcgtaagagttagggg

SEQ ID NO: 81 - DNA, 419 bp, Zea mays
aagcgaacgaggaaaggaagaacaagttggcttcgattgaaggctcgacaactgccgagtaccatctgcctgttctggcaatgacagccgatgttatccaggcaacttacgaagagtgcataaaatcgggaatggatggatacgtatctaaacccttcgacgaggagcagctataccaagcagtctccagattggtagtgggaacgacggattcggctgtttgatgttcaaaatacgatggacctgacttctcattcatcgaagtgaagcatcaccatcttgcctctgtccagctgactctatatcccttgacaatgggcctctgacatggcctctcacaagactagatgaaaaaagaagatgaaagtgccgtgagttaggtacgtgtcacacatgacatgaagttgctgcggcagccc

SEQ ID NO: 82 - DNA, 868 bp, Zea mays
attttgatccgtcattatcttgctcaaattctgtaactttcatcccaaagttcgccagaattcgtttcttttttattttgttaccagtagagcatctcctgatctacctcttcgtcgtgtttggtaaagactattgagctcaggtgtgttgcgttgtgcagagcacaggtggtgggatggccaccagtctgcaactaccgcaagaacacgatgactaccacccagctggagggcagcaaggaggatggtgatgccaagcagggtcaggggttcctgtacgtcaaggtcagcatggatggcgcgccgtacctcaggaagatcgacctcaagacttacaagaactacaaggacctgtcgaccgcgcttgagaagatgttcagtggcttcagtactggtgagatgtctcggggttactctctctctctctctctttcggatggcgcgtcagtgagtaattatgtttcgttttgatgtggatggtgttagaagtacatcaagaagcctttaaaaagcagcatactcctacttgattcctaggataagcaatagcttgaacttaccccgttatattttgagtaattgtaagattacaaacaatctggcaccccttgttttgttaatttttgggtgaactttttattcctcccaaaacaaataccctggtgattgttcagttattgcatccgtatcaagtctctcttagaaagatgttgtttcctgtaaggcaaaataagttttggctccatctttatgattattcgatgatatcttcgagtcctgggtattattccatagaaagctactaatcactatgagagtgacatcccctatatatttctgaaatttgtggagatctgtggtcctgtat

SEQ ID NO: 83 - DNA, 909 bp, Zea mays
cgctgaatccaacctaatgctgtacagaatatcctttacagccaagccgccaaccaagacgctgagtctaatgccatgtcctggtggatccaactatccaaacaacagatcaccccctttgagctgactgacgatcatgatgctgaaagtattggatgctggtcgaaggcttcaccctcttgctggctgtgaagtggaagacagagtcatgtaatcagtttgcttgccttcaaatcatacacctggtgtaaagtacagtttggtttgaatataaacaagtatcataaagtacttctttaaaattgtccaacgggggagtcagctgtcttttgcacctcagggtgcttcacacgtagctatatgatggtcactggttaactcatttacatagacaatttcagaagggataatctatgcaaaatctaatgatattattatgacccctgatccatttagaacaacatgagctgtactcctcctagatatgattacataagcatcttgatctatcaggcctttggtgagtactcaacactcaacagaaacctactaactcctatcgttctctgattaaacgagtgaacagttcaggacactgcagaagatttttttttctataagccaccgctattcaacaatcaacggttttgctaatcagatgtcacaaatgccaacatattgtcatccgaggatattccgtaaggtggacaagatagaaccagttatctcagaaaaaaaggccattaaaggatatctggtaataactacatcaccatccttctgtattcaagtattagcagaagagattgataatggaaggaaatcatccctgaataagcaccagtaatgggatatggtcatgtatcaaatgtaatttattaagcatcgcaagttttagaattagcaacc

SEQ ID NO: 84 - DNA, 827 bp, Zea mays
acaaaggaaagggaaagaaaatgacttctaggttttcacgtctccttttggttgaccaagaagagatggtcggtagagtgaatggccttgtgccatctcaattctttcgcgtggatcatacattgtctcatctcttatagcctgaagaatcgaatcagcaggacggtccctgtgcacatatgtaaacagaccaactcagtcaaatatcagaaaaccttagttcaatgaattattccaaactattgaaagataaagtagaatagctggcacacatgcaggggcagaaggaaccatgccaatcaagttatcggtatgtatgggttagtaatataggttactggcatataggtaatacgctgaaaatataactggtgtagagtatgtgacgttggtcttaggttctaacctcgtgatcagaatcctatgtagtgcttttaggatcgggcacatctcaaccggcgcaacagatctgttggcttctggatgcatgacacttaagctatcctgactaagaagctcataaaacgcatcaactgcagagacaccctgaaatggaacggcaacaggataattcatcacatgattcatttaggcatattcatgcagttctttgaagtttcgttgtcgaccaaaattaaaagggcatacctgaatggtcccttttcctttaatactgtcacccatttctaatgtcaattcacctttagctaacttctgcccataccatgcattacgacctttcaacaatgtgacataagtgtcagctaataagggtccagcaagtttttcaggttcttcttccagaaggtgtgtgatgtagatcatct

SEQ ID NO: 85 - DNA, 1867 bp, Zea mays
taccttgtttccccaccagagatagatagaacatctggggagtacttggtgaagaatggcatccgcacctttgcttgcaggcaagtactatctatttctcagcctttctcttgatacttttttatttacttcaatatcgtaaaatcacttagtttttctgagtcatctaagtcagcatgctccatttattttgaatcaacattatcaagtgtacttcgtacaatcttgtacatacctgtgaggagcactgaccttctggaaagatatcatttttcacttcacagaacatcaggaattcaagattcactcagttaattgatattttaaataattttgaaaattgaaatacaggaaaatatgtgtttttaaggcattacattttgcatataaatattcaatctcactaaaggaaaatgttttaagaacatttttctttagtgaaaaggaatccaaatgctttcgaattctgttgtgacttatctctattaccttatactgcatccgtactagtatatttgacatctgtagagaagagttcttttttctagggtaatcttctagctgcagtgcagtatgctgacattgtgctaacttaggctgatatttggttgcattgctctgcccatgatttgtgccctaatactgtatattagggctgcataatgttatttttggattgattcattgttgtatcatccttgtgcttgcaacatgatctacattttcccttctctctctctctctctctacttatgcagcaacattgttttgtgtgtgacagtgagacagttaaatttggccatgtcacatttttctggaacggtaaccgttcgggatactttgatgcaactaaggaggagtatgtagaagtacctagtgacagtggtattacattcaatgttgcacccaatatgaaggcgcttgaaattgctgagaaagccagggatgctctcctaagtggaaagtttgaccaggtaaataatttgaagtttctattagagcactctttcggtttccctgttgcttagcctagcgttgttacaggtacgtgtcaacctgccaaatggtgacatggttggtcacactggtgatattgaggccaccgtagttgcttgcaaggcagctgatgaagctgttaaggtgagagcaccaatgaaagttcgctgacatgtgtgttgtcttattatctgcattggaagttcgcttatacatcaataaaggttcttacagtagcacgcttcataggcctttgcctattttttaaccaagtgttcttctgaacagattattttggatgctgtcgagcaagttggtggtatttaccttgttaccgccgatcatggcaatgctgaggatatggtgaaaaggaacaagtctggcaagccgttgctcgacaagaatgaccgtatccagattcttacctcgcatacccttcagccggtgagtgcaatgccatttgaccccatgtcttttggttctctcccagcaaaatcatacccgtgttgattgcttggatgctaatgcctctgtaaaacttgcaggtcccggttgccattggaggccctggccttcaccctggagtgaaattccggaacgacatccaaacccctgggctcgccaacgtagccgcaaccgtgatgaacctccacggatttgaggctcctgctgactacgagcaaaccctcattgaagtggctgacaactaaacactggccacctgtgtccaattttggttatatgtagttctgagaatggacattcaataatttatgtttgcaagcacgttgctcaaactcaccaaaacatcgagggatgccttttgactttggcatttacagcattttcgtttggctttaatccttatcgg

SEQ ID NO: 86 - DNA, 560 bp, Zea mays
cgtccgcggcagcggccgcgtccaggtggtcgggcccgacggggtgcgcgtcctggagacgcgcgtcgagggcggcttcctcttcatcgtgccccgcttccacgtcgtctccaagatcgccgacgcgtccggcatggagtggttctccatcatcaccacccccaagtaatttgttgtctcgatcgatcgatccatcgatctttttttattgcgaattgcactggagatttgattgcacgtgaattaatgcttgcattgcattgcagcccgatcttcagccacctggccgggaagacgtcggtgtggaaggccatctcggcggaggtgctgcaggcgtcgttcaacaccacgccggagatggagaagctgttccggtccaagaggctcgactcggagatcttcttcgctcccccatccaactgagaaaataggccggaagccccacggtggagtcctctcgttaggtcgtcgtgcttagattaggttagctagcttgcctttaataaaaagagagtggtggtcgtcggcgtcggcttcggcggtctgcttcttcttcattc

SEQ ID NO: 87 - DNA, 496 bp, Zea mays
ccgtgttggttggatctatggctcggtgacggaggatgtggtcactgggtaccggatgcacaaccggggttggaagtcggtgtactgtgtcaccaagcgtgacgccttccgcggcaccgcgcccatcaacctgaccgaccgtctccaccaggtgctccggtgggctactggatcagtggagatcttcttctcccgcaacaacgcgctgctggcgagccgcagaatgaagttcttgcagaggatcgcgtacctgaacgtgggtatctacccgttcacgtccatcttcctgatcgtctactgcttcctgccggcgctgtcgctgttctcggggcagttcatcgtgaagacgctgaacgtgacgttcctgacgtacctgctggtgatcacgctgacgctgtgcctgctggcggtgctggagatcaagtggtcggggatcagcctggaggagtggtggcggaacgagcagttctggctgatcggcggcacgagcgcgcac

SEQ ID NO: 88 - DNA, 924 bp, Zea mays
aatgtgatatcatgatactcatgcacctgtaccttagccaatgcaggagtctgttaaagtctcaatagcattttgtgatgctcaccaacagttcctttttacaggattcatctggtatattctgggataatgacagtttagctggtcttttggctattgaacttaaagcagatctccttgttctactaagtgatgtagatggtctatacagcggtccaccaagcgaaccgggatcaaagatcattcatacctacattaaagataaacattacagtggaataacttttggggataagtcacgtgtaggtagaggaggaatgacagctaaagtgaaggctgcttttgtggcttcgaacagtggcacacctgttgttattacaaggtatgtattgcatttttcattctttatcgagaataaaaactgcccttcgttgctcatttatatgttcccatgtgattgtgatctatcaaactttccctgtgacatgcaaccaataataaggaatttagacaaaacagttgataggtggtgtgattaactacatatttggtgtagactacatttgactcaagtgtttatttttgggtgtagactacatttgactcgagtgtttcttacatctttaatgatgtgaagaattggttttcagaagtgaaatatttccttagacttttttctctctcgaacgcgcaggagagctgcacatcattatatttccttagactgttatgctgaatcctcgcttgtgatgttcacttatttttctatgttggattttatttacatataataaggtctgctgttcaaatccaaatacgccatctgttttcaatgtttgttcatggccttaggaaaatgtgttgcacattgtttgtctattgaggatatcaggagtgtagttattgctatgtttccactctccc

SEQ ID NO: 89 - DNA, 1140 bp, Zea mays
gtgaaggacaggggactcctggacagccttctcggcaggaacaagcacgacgaccaggagaagaagaaccagcaggaggaggaggagctcgcgaccggcatggagaaggtcacggtggctgagcccgaccacaaggaggagggacacgaggccgccgagaagaaggacagccttctcgccaagctgcaccgcaccagctccagttccagctcggtgagttcgtcgtaaaacatgatctgctgctagctagtttaattgactccgccttcggatcagtaagctaataaaccggcttctcactgcgatcgtggtgcctgcgcgcatgcagtcgagcgacgacgaggaagaggaggtgatcgatgagaacggcgaaattgtcaagaggaagaagaagggccttaaggagaaggtcaaggagaagctggcggcccacaaggcccacgatgagggcgaccaccaccagccgggcgtacctgccccggcgcccgcaccgcccgtggcggtggacacgcatgctcaccaccaggagggagagcacaagccgcacttcccggcgccggcgcctcccccgcacgtggagacgcaccaccccgtcgtcgtccacaagatcgaggacgacgacacgaagactcagaccccaccacaggcaccggaggaggagaagaaaggcctgctggacaagatcaaggagaagctacccggtggccacaagaagccggaagacgctgctgccgccgccgccgcgccggccgtccacgcgccaccgccgccggcgccccacgccgaggtcgacgtcagcagcccggatggcaagaagggcttgctgggcaagatcatggacaagatacccggctaccacaagagctcgggtgaagaagaccgcaaggacgccgccggcgagcacaagaccagctcctaaggtcgcagcgtgtgcgtgtccgtcgtacgttctggccggccgggccttgggcgcgcgatcagaagcgttgcgttggcgtgtgtgtgcttctggtttgctttaattttaccaagtttgtttcaaggtggatcgcgtggtcaaggtccgtgtgctttaaagacccaccggcactggcagtgagtgttgctgcttgtgtaggctttggtacgtatgggctttat

SEQ ID NO: 90 - DNA, 477 bp, Zea mays
gcaaaggtacagcgtaaaaactaagaggagagccagcaagctagcattttatttagtaaaatcgttcactcgcaggtacccaatcttctcagctttacacactcgccatcttgaggctgttgcccttctcctgcaggctcacgagtaggctgtcaaagctcttcttgaaggagtccacgccttccagctcaagctgctttccaacctcttcccagtcgatgccaagcttctccaaggcactgtatacaccttccgcctcagacacgttcgcatcaactgtccttgaaacggtgccgtggtctatgaatgcttgcaaagcttggtcgggcatcgtgttgacctgaaagtgcaccactacagagttatttttttgtgatgataagaaacaatgccagttcaagtgggaaactcgtcgtgacaacataccgtgtcaggtccgatgagactgtccacataaagagtgtcaggataagctgg

SEQ ID NO: 91 - DNA, 376 bp, Zea mays
ccaggcgaccaaggggttcaagaacaagatgctgctcggcaccggcggcttcgggagggtgtacaagggcgtgctctccgggtccaagctcgaggtcgccgtgaagagggtgtcgcacgactcgaagcaggggatgaaggagttcatcgcggaggtggtgagcatcggccacctccgccaccggaacctggtgcagctgctgggctattgccggcggaagggcgagctgctgctggtgtacgactacatgtccaacggcagcctggacaagtacctctacgacgacaggaccgccaggcccgtcctggactgggggcagaggttccagatcgtcaggggcgtcgccgccggcctgctgtacctgcacgaggactgg

SEQ ID NO: 92 - DNA, 820 bp, Zea mays
aaacaacaacttgtagttgtccacaacaggttaacagatcaaagaaggataggtgagcggcactactcatctcgtggcttccggtgacagatgatcagcccacgaaggaaaaagaaaaagggactcgcttgatttgcgttgctttgctttccgcgcaaggccgaaagcttaaggtcggggcaacgacacaccgagagcgacggagatataccacgctctgctgcttcatgatagctggaaggacatcagcatgacacgcatgccaataatgtagtagaagactagtttatttgtcacctactaggcagagagtgcggtggttccatgaaccaaccattcgtgcgtgcgtgcccaccgcacgaccacgagggggcatgcaacatatactttacaaaattcattcggttgttgacttggtttcaattcattgggttgggaagacaaaactaacatggatgcgttgcgtactcacaggaaggtgatggctcagactggtgagatccggtgcgccatggatcacatcctcgaggccgagaggaagggcgagatcaaccacgacaacgtcctctacatcgtcgagaacatcaacgtcgcaggtatcgataatcgtcactgctcagtgcaatgaaacggaaacagagtatgctatgtctgaagaaccaagtgagacttatcattcaactactgcagtccagcgctactacacaaacaaatagcactgcaatatcggaagatataataatataaggcacgtcttaatcaagtctccgtcagccaacttaattccgtccttaattaaccggcaacatactgagcctaa

SEQ ID NO: 93 - DNA, 683 bp, Zea mays
tgacctacaactcaaacaggctcgtcttcaatggccacgagatctacccgtcagcagtcgtgtctaaaccaagagtagaggttcaagggggtgacttgcggtcgttcttcacattggttagcaccagtccaacactactccacacagttagctctccaagttgttctatatatatatgtatcccggcgccccttcctttccctaatggccatagttcctgaatttccaggttatgacagacccagacgtcccaggaccaagcgatccatatctaagggagcaccttcactggtaacatctggcatttcctaccaacatctaggggaatgctgtgtgactggtatatgtcctttacatttgcaggatcgtgactgatatacctgggacaactgatgcctcattcggtagttttttctcccccctctgctttgtggttaattagtcgttccagttgttcttggagctagttaattagtagcaggcattttttttcagggagagaagtcgtaagctatgagagcccgagacctggcattggtatccacaggttcatctttgttctcttcaagcagaagcgcaggcagcagcagactgtagcggcggtgccatcctccagcagggaccatttcatcacgcgtcagttcgctgcggaaaacgatcttggccaccctgtagccgctgtg

SEQ ID NO: 94 - DNA, 765 bp, Zea mays
tatgcatgatttatgcccgccaaacagacagaaaacgcaacaaactacaaccatttacagaccggagccaagtgaacctaacttgttaacatcatatgaaggaacatcctaaacgagcaatgcttactcaaatttactgctatgctacttctattgctgttaatgaggcagtcactcacaggctgctgctgactggaaagccaggggaaattagcgttctggcttcaggtcacgatcaatgtactgcctcacagcctcttggtttacatggaaaataaacctcatgtcctttatctggaaagggggggaaaaaggtagctaaattagtacagcatgaagatacttaattaaatgcatcagtgatatctcagtcaaataacaagggaaggattgtcaggtatagcaaaggttaacttgtcaaaaagtaattgtttcatgtctgcttacatatcaccatagtatcattcgtactgtttttagatactctataaaaccccaaaataacataatggcaagaagtaaaacttcaagcaccctctaccagtagaaccataaactatgacaggatcacaggaatagttacaaaaactgtgcattgactaaccaccaggttacagattcattaaaaaatgaaggtatactagaacggggaagtattggtacctcgattaatgagtctgagcttaggttgatgcgtttgcagcttggtatttccttgctattaacaaagattggacattttccagtgttcttaatatgaaaata

SEQ ID NO: 95 - DNA, 770 bp, Zea mays
agcatcatggagtacggtcagcaggggcagcgcggccacggcgccacgggccatgtcgaccagtacggcaacccagtcggcggcgtcgagcacggcaccggcggcatgaggcacggcacgggaaccaccggcggcatgggccagctgggtgagcacggcggcgctggcatgggtggcgggcagttccagcctgcgagggaggagcacaagaccggcggcatcctgcatcgctccggcagctccagctccagctcggtaattacgactctggatacttctttcttttgtgtgcgcgctgcttcgtcctatatataataatacatgagttaggcttagtaataatcaattaatttaatccgtgggtttcgtgtttaagtcggaggacgacggcatgggcggaaggaggaagaagggaatcaaggagaagatcaaagagaagctgcccggaggccacaaggacgaccagcacgccacggcgacgaccggcggcgcctatgggcagcagggacacaccggcagcgcctacgggcagcagggacacaccggcggcgcctacgccaccggcaccgagggcaccggcgagaagaaaggcattatggacaagatcaaggagaagctgcccggacagcactgagcggcgcctatacgtggctgtgctgtgctgtgctggcgcgtcaaagccgtactcttcagcgttccatagataataagataaacccatgaataagtgtccctaccctttgatcatgtgacagggacagggacaggga

SEQ ID NO: 96 - DNA, 422 bp, Zea mays
aaggcaacattctgaagatgcagcgcaagcagaagccatgcactcccctcccctccaacaagcagagtcggtactaccggcctcgggtcaaggtatgcgccagaacccgactccttgaggcgatgttccccgcaggggcaagagtctctgaagctgcctgtctgtctgtctgtgtgtgttctcgctttctttcgcaggggaggtttgtcagcaaggcttgtttcctccagcgacagcaagcgttagagaaggagagctagagaaagatggatcctgctccaaggcgcatttctggggctctcttggagaagcagcagagcttctccgttttcatctctgcggcggtacagtgcggcagatgtagagatgcctgtagagtggtgcttgtgaacctcaattctcagtttcttctatccattcca

SEQ ID NO: 97 - DNA, 553 bp, Zea mays
cacaaaagagaaggctctcaaggtgaactagaacagaatctcccgacggccggggctcaaaccagctcatcctcggcgatatctcgaggattcctcaccagctcgagcatgctcacgacctcacccatgccaggccggttcgacggcacctgagaggtgcacacaaggcccagcttgatgaccggcagggcctcgtccatggggaactcgccgcgcagccgagggtcgacgcagtcctctggcctgccttcctccagcgcgcctctgaccaggtcacacaggacaaccacgtcgtcttccaagtactccacgggcctcctgcccgtcaaggcctccagcagaagcaccccgaagccatagacgtcgcatttctcggtgatcttcaccgtcttgcacgcaaactctggcgccatgtacccgagcgcgctctggaccttactgctcaggacgtaccggtccagcatcggcagcagcttggcgaggccgtagtcacccacctttggctcgccgttgctgtccagcagcacgttgcttgacttgagattgtagtgga

SEQ ID NO: 98 - DNA, 612 bp, Zea mays
gcattcattgctgatgtttttgaatgactcttaggacaagtgtggctacaccggagcatgtcgaagaggcattcagactgttcaatgtttccaccgttgatgctgcaagatccggaatcaatgagcatttgaacctgtcaccggagatcgcaaacgaaatcaaggttagtatttgcatcccagggtatacaaaattcagctattgaaccttgcattttcctgaacggctttcatcatttttttttcatctgacagcaagcggaggcacaaataaagagaagaatgggcatcggcagccacatatccgagcgacggctgattgatgatctaaaccggatggggatgaatgaatccatcgtaggaaccctgtcatcgaatcttagaactgaaactatggttttcaagtaagacccgttcgtttttctgacaatatcttgcacactttgtttcaggtcagaagagcccttctgatcatgcatcaaagggacgaggtggagtacaagagagagcgccacgtgatcgtccgaaaggcttgaggtggagaggccagtcagattcacggcatacaacgtacactggaggcggtccttcctcttcggacgtgtgtatacc

SEQ ID NO: 99 - DNA, 664 bp, Zea mays
ttcctctataagtacccgccccacatctgcgccattttctcatcgcagaaatcctccgcaacttcacagcgtatcatcgttttccatcgctcctactcctatcatccagaaaatctgagcggtattgatggcgcccaaggcggagaagaagccggcggcgaagaaggtggcggaggaggagccctcggagaaggcggctccggcggagaaggcccccgcggggaagaagcccaaggcggagaagcggctacctgcgggcaagtccgccggcaaggagggcggcgacaagaagggtaggaagaaggcgaagaagagcgtggagacctacaagatctacatcttcaaggtcctgaagcaggtgcaccccgacatcggcatctcctccaaggccatgtccatcatgaactccttcatcaacgacatcttcgagaagctcgccgcggaggccgccaagctcgcccggtacaacaagaagcccaccatcacctcccgcgagatccagacctccgtccgcctcgtcctccccggcgagctcgccaagcacgccgtctcggagggtaccaaggccgtcaccaagttcacctcgtcttagccgccttgttgtaggcgtcgttgttgtctgcttctcaagcaagcactgtcatgtgccgcttctcatggcagt

SEQ ID NO: 100 - DNA, 680 bp, Zea mays
aaacaacacagtcatctgatcgtcataaaatgatataatctgtctataccgcacccaagtgtttcagtctttcagagttccaaaacgttcgaatcttttctttagccatcttcttcctcccgacgccgccgcggctatgaccgcgtatgagttccaacactcgagtgaggtgtagagtgtagacttaccgaaatgatatgtatacttgtagtaatacatgacaaaacgacggttaattcttgtgtaacaatgcgatacgagcagggccgatgtactacaacggcatgtaccatctcttctaccagtacaacccgcacggcgcgctctggggcgttggcaacctctcctggggccactccgtttccggcgacctcgtgaactgggccgccctggacacggcgctggacccgacgtcgcccttcgacgccaacggctgctggtcgggctccgccaccatcctccccggcggcaccccggccatcctctacacgggcatcgacgccaacggggagcaggtgcagaacgtggcgttccccagggacccggcggacccgctccttcgccggtgggacaagcccggctacaaccccgtcatcccgctccccgccgacgtcccgggcgacaagttccgggacccttcgacggcgtggctcggccgcgacgggctgtggcgcgtcgcg

SEQ ID NO: 101 - DNA, 935 bp, Zea mays
ctgtcatccatgtccaggaggtctgttgctgcacacccttggcatgatctggagataggtattgtacacgctctagcttgacaaatggtcagccgttgatctctgctatttgcaaccagagcttaagttcatcttggattcatgcaggtcctggtgctccaaccatattcaactgcgtaaggccaccctgtcatgcttgactggtcctcttgtgatatgttcatgttaatagcatgatgtcttttgttctattggaaaataaaaagtctccctggactctaaaatcaatgcctgtgaacacatgaactgtttgtgtcacccatgttcctctgctccttggcactttctgatgcatgctcaaatgcttaagaaagactcatagaagcgactcctattcctatgccaggtcattgagataccaaggggcagcaaggttaaatatgaacttgacaagaaaactggactgatcaaggtaaagcaatgttgttttcctcccgctgaagtcttattgtgaagctatatttcttgccagttctaatatttactcctttccgtttcaatctgtgtgcatgtgcaggtggaccgtgtgctgtattcatcagttgtttaccctcacaactatggattcattcctcgcacgctttgtgaagacagtgatcctttggatgtactggttataatgcaggtatgcttcttttttatatatatcattgggattcacaaaatggtacatcagtagtgatctgagtatccttgggcataagttgagctaattttcaaatcttgtcattttccatttctgggaatggtcgagaacatgtctataaactgttacttccaagcatgtaggagccagtcattttccatttctgtttatagttgcctagtcgggaacatgtatgtaaactgttacttccgtgcatgcaggagcctgt

SEQ ID NO: 102 - DNA, 805 bp, Zea mays
ggatccatacaaggtgcttttttttcgatttagaattctttcttcatcgattttgccctatgtgctagatcctcaaatcaattccgcatcttgtttccgcccttgattgatgcattcgctcgtctgacttgattgatgcgctcgatctgggggactcttcgttcttgcagcaccgcccgtctagtgggagcaactccagcttctggaccaccaactccggcgcccccgtctggaacaacaactctgccctcaccgtcggacagcgaggtcagaccacaacccctctctctgtttatcctgtagctgacatgctgctgccttcatttgtctcgtctctccatcccggtttcattttcccttgcacgatcctgtatgtactcactatgtatgtagcatatatgttcttgatttgtgcgagacccatccgaggcataaatgatctgttctagctttgctttgaggcctattattgcaccgtggaagccagaggatttcgcttcccatccattcaaagcttgcatcttgatgtgcttttaattaatttccagtgactaattttgcctgctctgtacatgcgggttgtcgttgattcacctgtccgaatatcgtcaatgaatttgagacttgcccaaaggacttattccttgtatcagctgtaaggtgaagcttttgtcctgatatttttgccagtcgctgtcgaaccattacgttacttaagggaaagaaagcacattcccggtacgaaatgccatcatggagtcatagtgataatcctaggtgagggacacttggagagtagtaaagt

SEQ ID NO: 103 - DNA, 1582 bp, Zea mays
gtacctcctattcttagccagctagcgagagagaccaaatcctggcctcacatgagatcgactggttcctgggctccttctctcctccccccgttaagttgcccgtcggaggaggatcctgagcacatcgatcagtcgcgtgtctaggtttcctctctcaccatagcgcccgctctgtcgcccttcgttcacctctccttcctctcgtccctgcctgccagggagaggggaagtcagaggcacggagtggcgcagagcagacgcccgtgaaccattgtagctgtccctgtcgtcgtcgtcgtcaacgaacccacacaaggaaaggatggagaagaagccgaccatcctcatgaacaggtacgagctcgggcgcacgctcgggcagggcaccttcgccaaggtgtaccacggccggaacctcgcgtccggcgagagcgtggccatcaaggtcatcgacaaggagaaggtgatgcgcgtcggcatgatcgaccagatcaagcgcgagatctccgtcatgcgcctcgtccgccaccccaacgtcgtgcagctgcacgaggtgatggccagcaagagcaagatatacttcgccatggagtacgtccggggcggcgagctcttcgcccgcgtcgcccgcggccggctcaaggaggacgccgcgagaaggtacttccaccagctcgtcggcgccgtcgacttctgccacagccgcggcgtctaccaccgcgacctcaagcccgagaacctcctcgtcgacgagcacggcaacctcaaggtctccgacttcggcctcagcgcgctcagggagtgccagaagcaggacggcctgctgcacaccacctgcggcacccccgcgtacgtcgcgccggagatcatcaacaagaagggctacgacggggccaaggccgacatctggtcctgcggcgtcatcctcttcgtgctcctcgccggctacctcccgttccacgacgccaacctggtggagatgtaccgcaagatcagcagagccgacgtcaagtacccgcagtggttctcccctgagctccggcggttgatgcccaagctcctcgaaccgaacccaaacaacaggatcacgatcgagaagctggtcgagcacccctggttcaagaaggggtacaggccggccgtcatgctggcacagccgcacggctccagcagcctcaaggatgtccaggtcgccttcagcaacgccgaccacaaggacagcagcagcaaggtggaacagccggcggacagctccttgaagccggcgagcctgaacgcgttcgacatcatctcccactccagagggttcgacctgtcaagcctgttcgaggtggaccaagagcagaaggccagcaactcgcggttcatgacccagaagccggcgtcggcgatagtgtcaaagctggagcagatcgctgagacagagcgcttcatggtgaaaaaacaggacgggctggtgaagctgcaggggtccaagcaagggaggaaggggcagctcgcgatcgacgccgagatcttcgaggtgacaccggcctttcacgtcgtcgaggtgaagaagtcggcaggcgacacgctggag

SEQ ID NO: 104 - DNA, 741 bp, Zea mays
gcaatgtgaatgaatatatgacgcaccattatgttatgtgtgacatattttgatttctatacttctaagtattctctgatcatctgggacgtgtaaacataaaaagataataaactaactgcattcgagatcatgaccagtaataacaaacaaatgtaatctgcagtgagaacagataagtggccacataaccaaaaccttgagtctgcacagcatcttaattgtcacttaacacaagaaaacaatttagacagttataagcaacatataacattgaccattgatcatttaggttaacatggggacaagacataattgattgctaaatctatctgtaagctttattaatcttataattcataattacaatgagttcattgcaaccctcaaggtgtaatgttacagcaagtcaaccacagcagcacagaacaagaacatgttgtagacctaaggttttagtctccctttgaactctattactcagatatagagtatatatctaacaaaaatggtacggaaaagcatacctaagaaaccacaagccacagaattgatgtagcttcgagcttcaattgaatccagacctaggacaattatgtggaactgactgtagaactctatctctttatcttcaatcctgcaaaaatgaggaactatgttcaccccattaactcgctccataaccctcttcgctgctacttcagccttggacttcccaacatcttgaactctgtacagcag

SEQ ID NO: 105 - DNA, 628 bp, Zea mays
gagaagcaacatgacggcaagctcagtggctacattcgaataaggagcaagacccagggaattgcactcagcttaggggacaagatcactctcaagcagaaaggtggcagttaactgtgacaagtaatcgcagttgtatcatcatttttcgcatttaggaaatccacgtgccagagagagaccagtgccgtggcattgaactgagtataaatgcttttttgtacaaaaggatcgatcaaggagagagataagaggacagttatgaggaagtcacgaagttgtcggtcgaagatatatgttgctgtagtaacgaagctgttccaaacttccttgaaatagttgtgaagtttatgttgatttctcgacaggtagttcaattgtgatcttgtactactattatgaatccctcttgttttaatgttttatttgcctttattttagttgtctggacttggaaacagaagcttggaggcggtgttgtcacgttatttttgtagagatgaattggagctcattttctgttgcatatagatttgccaattgtgttagggtacttttatggtgtttatttaagaaatgaggtagtccattatctttttactcagtttctttggtttgtggaataaat

SEQ ID NO: 106 - DNA, 1084 bp, Zea mays
atagtgcaaatctgagtgttaaccataataacacaaatctgagtgttgcacagagaaaaggataacgcatgtagcagatcaacatatttataatcatagtgcatcgcagcccaatattgaaacagataaaaatacattaaccagtagagagttgtaccaagagagaacagaacttacttcctgagcctgagctggggtggcgactttgccagttccaatagcccagactggttcataggcaagaacaacgttgctccagtccttgatcttctctgtaaaacaaacagccatttgatccattcagcctgatttttcgtatagggtcaaaaaacttggtaacttcaaagcaaggcactaaatgttcacatgaacaaaacaaagggcagacccagctcccacatgaatgtggggtctttcccccacaaatgcggaaaggaaaatccagcatgtaaattcatccaagcaacagaaacaaaaactcggccagggaaggaaagaccgccctcccggtattctattaagaagagaccgaaacatggtcccggccgaaaaaatccccgaaccctagccccccatcactagttggccgacatcgcgcactctgcaaatgcccagccggagggtggggtgcatgacataacccgagggcgggcggggcacaacgaagggattttttaaccaagcccgaaattcgcccccaagggggatcgaacccgggacctggaggtgctacttggaagctttaaccattacgctaaaggccctttcgcagcgacagaaacacacataagttgattcctaaactaaagctgttacagaaaaacagtaatgtccgaactccggatatgtagattatctaacagaactgatcaccagaagcaaagggcctgttcagtttgggtttcagctgctgtggctagctgcagctagcttatgactacagtaactctactgtgacacctgagaggcagcagccaacgactgaataaatgccagacgaacaatctcaaccaaaagatgtatagctacatttatataatgaaccaacaaggcagcaactcttcattaccattaaaaaactaac

SEQ ID NO: 107 - DNA, 929 bp, Zea mays
atcaagagcagcagctgctttgctgagaaacaggctgaccccgcatttgcacagttgcaggcctactagcaccacttgcagctggttgacttgccatcctatccaacaaggagaatgaagaatgattaggtgctcccgtatacagataaacaatagcaaacatagtgatcatgggattcatggcttatttttcactttgaatcatatgcaatattatgttgcacagtgttctttgtttgtactcagtccctcaataaaagagggcctccatatgttgacatactatacttgatgactccaaaaggaatgagaaaatgctgccacaaaaaagtctacaacacaaatgatctagttacctgttctttatctcccctgccatggtcatgaatgccttctccacatttgttgcatccttggcactagtctcaaggaatggtattccgatgtcatcagcaagggcctatgatgacaagcaacatgcagccaatttaactatcatcccggttgaaagaagcatgtccagtaaaagtaattaatgcagagaaatattaccttgccagcctcgtaagaaactactctgttctcagccaggtcacacttgttccccaccaaaagcttgttcacattttcactggcatacctatcaatttcattcagccactgcttgacattgttaaagctctcctggtcagttacatcatacacaacctatagaaatacaaaagtttaaacaagactcagattaacaaagatgagataatagcagataggaaaaaaacgaaataagaaaaagaaagctcacaataatgccatgagctccacggtagtagctgcttgtgatggtcctaaagcgttcttggccagcagtatcccactaaatcagaagaatgtggagaaacataagtgtcaaagcttctaactgttaggaa

SEQ ID NO: 108 - DNA, 850 bp, Zea mays
ctcgggcaccggaattcccccctgtagatcttacggtacatcgccatgaggttctggtcgtggaaagggaggtagccagccatgagcacgaacaggatgacaccgcacgaccatatgtccgccttggcgccgtcgtagccgcggcgcgcgagcacctccggagcgacgtatgacggcgtgccacagaaggtgtggaggaggccgtcggggtggaactggtcggcgaccgccgagaggccgaagtcggagaccttgaggtcgccgcgctcgtcgacgaggagattctcgggcttgaggtcgcggtggaagacgccgcgggcgtggcagaagccgacggcggagatgagctgctggaagtacctgcgcgcggtgtcctccttgaggcggcccttggcgacgcgcgcgaagagctccccgccgcggacgaactccatgacgaagtagatcttggacctggtggccatgacctcgaagaggcggacgatgttggggtggcgcacgcggcggaggatggcgatctcgcgcttgatgtgcgggacgaggccgttgcgcagggccttctccttgtcgagcaccttgatggcgacggtctcgccggtgtcgtcggcgtggcgggcgtggtacaccttggcgaaggtgccgtggccgagcaggcggcccagctcgtagcgccccagcaggaggcccccgcgcttggcgggccccgaggaggaggccggccgccggggctgcggtgacgcgtcccacgacggcggcggggtggcggccatcaggtagaggaggaggtcaggcgcgcggagaaacggagcggaaggcagaatggccgattaggtggtggtggtagcgaggg

SEQ ID NO: 109 - DNA, 606 bp, Zea mays
gccaaacaagcactcttctagttcttccgtttctcactttctcttcctgagaatctcccctttatatgaataatataaatgtcacataagtaaataaacaaataaatcaatcaatattactacgaagctgtcctcaccgccttctctctccctccgaatccaaacgcggacgcaaatgttgctccacgccggtccctcgttcctgctcgcaccacctccgcgctttgccgccgctccgtcgtcagcttcgccgaggcgatccaggacaccgcaatcctcgccgccgacgtcgcatttcgcgcgccccgctgatcccgtggcccaaagggtgcgtcccgtcgcgccgaggccccccatggcgacggcggaggagggcgccagctctgacgtcggcgtcgccgtcgccgagtccgcacaggttcggccgccactgcccctcctcacattccagagtttacgcaattattatcacttgggccactcgtttgccaatgattacgcgattacgcctaacctgtcggtcgggtctacattgtagtcacactcacacgaatgcccccaaccgtttgtgagctcgtggtgatgatctgtgttccacctgcacca

SEQ ID NO: 110 - DNA, 710 bp, Zea mays
agcatgaccagaagcagagcctgatggacaaggcgaaggggttcgtcgcggagaagatcgcgcacatccccaagcccgaggcgacgctggacggcgtgacgttcaagggcctgagccgggagtgcatcacgctgcacagcagcgtgaacgtgtccaacccctacgaccaccgcctccccatctgcgaggtgacctacacgctccggtgcgccggcaaggaggtggcgtccggcaccatgccggaccccggctggatcgccgccagcggctccaccgcgctggagatccccgccaaggtgccctacgacttcctcgtctccctcgtcagggacgtcggccgggactgggacatcgactacgagctccaggtcgggctcaccgtcgacctccccatcgtcggcaacttcaccatcccgctctccacctctggcgagttcaagctccccaccctcaaggacttgttctgatctagtagtagctcgcttgccttgtgttctgtgcgggcgcgcaccagcgatctgtacgacgagcttttgcaaataaacgacgcagctcctctgttctatatatctcaatgaatgcctaagctaaggggatggatggtttaatttgactgcaaataaagagctggatttcgttcaggttcctgtctctaagctggatttcattcgggcatccaccatgatgtggatgtgcctgccgcgtccgtc

SEQ ID NO: 111 - DNA, 838 bp, Zea mays
acgacgatggcggcgtaccccttggggatctccgcgacgccggagaagccgaacttggcgccgatgaggctgcccacgacgatctggcacgcgagcatctgggtgccgccctgcaggaacagcttgcggcggccgaggcggtcgacggtgacgatggacacgaaggtggcgaagacgttgacgaggcccgtgatgacggcggacatgagggaggcgtcgtccgcgaagcccagcgtcttgaagaggaccggggcgtagaacatgatgacgttgatgcccgtgagctgctggaacatggggatggcgatggccatgacgagctgcgggcggtagcgcggcagcaggatgttgcgccaggggtgcgccaccagcttggactcgtcgctggcggccaccaggtcgctgtactcctcctccacgtcgtcggtgccccggacgcgcttgagcatccgcttggcggcgtcggtgtagccgcggtcgatgagggagttgggtgtgtcgggcaggaagagcgcgcccacggcgatgatggccgccggcacggccgcgagcgcgaggctgacgcgccagccccagccgcccctgatcttggcggtgccgtagttgatgaggttggcgcagaggatgccgatggtgaccatgagctggaagccgatgttgagcatcccgcggaggcgcgccggcgccatctccgagaggtagacgggcacggactggttggcgaagccgacgccgacgccgaggaggacgcggccgaggatgagcatgcccacgtccttggcggcgccgttgagcgcggcgccgaccaggaacgtgacgccgccgccgaacatggacc

SEQ ID NO: 112 - DNA, 821 bp, Zea mays
ccagttcaagacagaggagatgaccaacatcatgaaggacttcgacgagcccgggttcctggccccgaccggcctcttcctcggccccaccaagtacatggtcatccaaggcgagcccggcgctgtcatccgcgggaagaaggtactgatccgtcgtcgtctatgctccccctctcgatctcccaatataatgcacgtcgatcatctttctcttgtttccctagggatctggaggcataactgtgaagaagacagggcaagcgatggtggtcggcatctacgacgagcccatgacccccggccagtgcaacatggtggtcgagaggctcggcgactacctcgtagagcaaggcctgtgaatggattcatttaacctcgctcgctcgcttgtccatggttcgagcatccagcagcaacgataccaacatcagcattatttaattggtagcctcctctagctacgcacgcattttagtcccctacacgcccttggattgtgcgtggctctgttaatcatctctcatccttcgtctgccatttctcccctgcccgtcgccgatcaccagagatttttgttccttgttggtaccatgcattttggcaaataattttgtaattccacccccaaattaaagtttggttgtcgtatggtttgtaaacccagaacaatatatatatgtgtgtgattgaactgttcctgtctattctttttgtaaacgggaatatatatgtatgcattttgtgtgatgcatgccttccagggcgacgactaattaatgtgcaaccagtcctccatccatgtatggtgaagggctaaaggc

SEQ ID NO: 113 - DNA, 652 bp, Zea mays
gtggaagccgccgcggctttcttgaacaaagccgtcaagccagtgcttgtaggtgggccaaagatgagggtgtccaaagcatgggaagccttggcagagctggcagatgcctgcggctatcccgttgccgtgatgccttctgcgaaggggctagtgccagtgcaccactctaggttcattggcacgtactggggtgcggtgagcactccattctgtgctgagatcgtcgagtctgccgatgcctacctatttgctggccccgtattcaacgactacagctcggttgggtactcgctgctcctcaagaaggagaaggccatcattgtccaaccagagcgggtggtggtcgggcatggacccgcgtttgggtgtgttctgatgaaggatttccttcatgcccttgcaacccgtctgaagaagaacactgtcgcgtatgagaactaccgtcgaatttatgtgcctccaggcgaaccactttcatctgaacctggcgagccgttgagagtgaacgtgctcttcaagcatattcaggcaatgctgtccggcgacatggctgtcatcgcagagactggggactcgtggtttaactgccagaagctgaagctaccggaaggatgtgggtaagctcctctttcgaatcatgattttgctg

SEQ ID NO: 114 - DNA, 646 bp, Zea mays
ccaacagatgctcaggtgaaccagtccagcagcataggcttctaaacctactattaggggaaaaagaaataacttatggcgtcgaccacaaacacactgatgcacgagaagtatttctagctgttgttatctgtgaggttgatcctgcggcggcggcgggctcgacacgatgtgaccataaacgaactggttccacgtgtccggcacgccggggaggcaccagtggatgcaatccgcgaacttcctcgggttcgccttctgctcgggcgtcaggagcttcccctgccgcagcgtgtgcacggaggtgtgcgcgtccttgcggatctccgacagcgcggtcacgtcgacgaagcgcaccggcaccttctccatcgacctcgtcacgcgctgggcggccgcgaagaggtcccagtccgtgcccacctccagtttcttcgtgtagttgatcgccggctgcgtctcggagaagcattttacggcgttggggctgccccagccttcactcctggaccacaacaagacagtgagtgactgtggaggggcagaaattctgcatatcaagcaaggtacggatggatacttactgcatatgtaccggtgacacgctcatgaataggaccgtgcttctcttgggatcaatgtgcgc

SEQ ID NO: 115 - DNA, 603 bp, Zea mays
ggatctggacaatatttcacaagccaaaaagacaaaaaaaaaaaaaatcaagtacctgtcttccatccaagcaacactgtacaggtctcccaaacaagtgtcatactccggtggagggctcgggaactcgccagggcagtacgtcccccagctgctctcgtctgcatttgacgcggtggtcgcatacacattgatgtcattcggcaggaggccctcaaagatgctcccagattcgcatgcttcaaggtaaaagacctacaaaaggtgaaagaatacgcatatacctcaagcccttgcttgacatatcacaaaatttcagagcagaactgaacaaacagctaacggtaccaggcttttgtaggtcccggcagcatgcttcttcttcaggacatctacgaggtcatcaccatagagatatggatacgtaggcattcctgaattttttacagagtaagtaactgtgtctattttggttctacatgcatgtacgaactgatattttatctaagaaacatctaatctgaatgaaatcagtagcaattagttgcgagtacagaccaaggacaccaggacccccatggtcactgtagaaaacaaagatat

SEQ ID NO: 116 - DNA, 841 bp, Zea mays
taactgctaataactataggcgggattatcatctgggttcaaatatttggacttatgtgctcctttgaggcggcgaggcagccacacccacacgcagtggcctgtggcgcctgggcggtgagtccgcctatgactgcgaatgttataattttattgggcatccttttagttgattgaattggttgtagcctgaaccttatctaccattttatctcccctgcttgtcgtgttctatgtccctgttcagcagctataccacagtcttttatgctcacagaggcagacattagtggcttgaagtgcagccaaacggcttaggtttatctatctcttctgagatatgaaatgggacattgtaggtttatgcatattcagccacctttgctagttattatgtgattttgtaaatttcctgagcctgcgactaaattatttcaacatatttagtaatgcgctgggagtatatgcagaacttaagtaccttttctgtttgttttgtcaacaaagtgagcaaaaaacaatgctttgttatgtgtggccatgttgcatgagtgaagaagcacgtgtttctttcttttcacctgaaaagtaaaatagttctgcaagcagaatctctagttatggaatgttatttctgaatccgcagttcacatcatgttcagtcaagtactagcactgacggttgcttcctttttgatatgtgcagaaagcacttgcaggtctgagaagaatcaatttagatgggcttcgatggcgcgtatttgatgctaagggtcaggttaggattgtttttctagcttgagtagcatggatgaacttatctcaagaaggatagaggcta

SEQ ID NO: 117 - DNA, 459 bp, Zea mays
atcaacgtgcagaacaagaactcgtcctacttcgtggagtggatccccaacaacgtgaagtccagcgtgtgtgacatcccgccgaggggcctgtccatggcgtccaccttcgtcggcaactcaacttccatccaggagatgttccggagggtgagcgagcagttcactgccatgttcaggaggaaggctttcttgcactggtacacgggcgagggcatggacgagatggagttcaccgaggccgagagcaatatgaatgacctcgtgtcggagtaccagcagtaccaggatgcgactgctgatgacgatgaggaggccgagtatgaggacgaggaggagccagctgatggcatgtgaggggaggctgttaaatgtgaagcctggtgatgtcccctttcgtgttgtcgccatgttatactagtacactagcataccaccctcgtggcccattccgtcgat

SEQ ID NO: 118 - DNA, 24 bp, Zea mays
ctagggtcctgctacaagagatcg

SEQ ID NO: 119 - DNA, 17 bp, Zea mays
ggtccagcccagtcgcc

SEQ ID NO: 120 - DNA, 20 bp, Zea mays
gaagagaagcaccctggacg

SEQ ID NO: 121 - DNA, 27 bp, Zea mays
  misc_feature (18)..(18): y is c or t
aacggacaatcaaatatytgttgtcag

SEQ ID NO: 122 - DNA, 26 bp, Zea mays
tcaacaaatcagaacacactcacagt

SEQ ID NO: 123 - DNA, 25 bp, Zea mays
caagcgttccagtgttattgagtct

SEQ ID NO: 124 - DNA, 19 bp, Zea mays
ggcgcataggacatcgtaa

SEQ ID NO: 125 - DNA, 25 bp, Zea mays
gtgattaaaggcttccgagtaacac

SEQ ID NO: 126 - DNA, 20 bp, Zea mays
agtcgttttccccacccttt

SEQ ID NO: 127 - DNA, 20 bp, Zea mays
cacacgatgttgccccatac

SEQ ID NO: 128 - DNA, 17 bp, Zea mays
agctgacgggcggatgt

SEQ ID NO: 129 - DNA, 21 bp, Zea mays
tgccattgttgaacacgaaca

SEQ ID NO: 130 - DNA, 21 bp, Zea mays
catgcctcagatcgtcaaaca

SEQ ID NO: 131 - DNA, 23 bp, Zea mays
cgccaacaagggaagaaattaaa

SEQ ID NO: 132 - DNA, 21 bp, Zea mays
aagaaagacaatgttggtggg

SEQ ID NO: 133 - DNA, 21 bp, Zea mays
ttcaacaacctgcagaacttg

SEQ ID NO: 134 - DNA, 23 bp, Zea mays
gccataccctgcagaatcagttc

SEQ ID NO: 135 - DNA, 21 bp, Zea mays
ccatcaggtgagcagcatctg

SEQ ID NO: 136 - DNA, 21 bp, Zea mays
cattcgcagccattcctacag

SEQ ID NO: 137 - DNA, 24 bp, Zea mays
ccgatggattggactcctgtttag

SEQ ID NO: 138 - DNA, 23 bp, Zea mays
tgggcagaaactgtggaagaaaa

SEQ ID NO: 139 - DNA, 22 bp, Zea mays
tgagggtgaggtgattctcgat

SEQ ID NO: 140 - DNA, 19 bp, Zea mays
tcaccgagttgagcagcag

SEQ ID NO: 141 - DNA, 15 bp, Zea mays
cggctgacgctgctg

SEQ ID NO: 142 - DNA, 26 bp, Zea mays
aaatgttgtgattttcaggccaagac

SEQ ID NO: 143 - DNA, 20 bp, Zea mays
tgctgtgagtagtgcttgca

SEQ ID NO: 144 - DNA, 22 bp, Zea mays
aggtcgaagatgaggacgttct

SEQ ID NO: 145 - DNA, 20 bp, Zea mays
gtcatgcgcatcatcaacga

SEQ ID NO: 146 - DNA, 24 bp, Zea mays
ggacttgtagtagacgttgacgta

SEQ ID NO: 147 - DNA, 16 bp, Zea mays
cgggctcctggtctgg

SEQ ID NO: 148 - DNA, 26 bp, Zea mays
gtgatcgctctgaatgtttaatgtgt

SEQ ID NO: 149 - DNA, 25 bp, Zea mays
ttcaacacctcagtacatcgctaaa

SEQ ID NO: 150 - DNA, 27 bp, Zea mays
gctttcgaatgtgttcatgatgtaagt

SEQ ID NO: 151 - DNA, 17 bp, Zea mays
ccccagccctggatcac

SEQ ID NO: 152 - DNA, 19 bp, Zea mays
tgatggaactgcacaaatg

SEQ ID NO: 153 - DNA, 18 bp, Zea mays
caccctgctcaaggtcat

SEQ ID NO: 154 - DNA, 27 bp, Zea mays
aggagaaggatgtggacttaattagaa

SEQ ID NO: 155 - DNA, 24 bp, Zea mays
tagatgtcctcatcctgaaacacg

SEQ ID NO: 156 - DNA, 22 bp, Zea mays
ccctggtaactcgtcccctaac

SEQ ID NO: 157 - DNA, 22 bp, Zea mays
gatgccctgctgttcttcagtc

SEQ ID NO: 158 - DNA, 24 bp, Zea mays
caagcagtctccagattggtagtg

SEQ ID NO: 159 - DNA, 25 bp, Zea mays
catctagtcttgtgagaggccatgt

SEQ ID NO: 160 - DNA, 25 bp, Zea mays
tgttaccagtagagcatctcctgat

SEQ ID NO: 161 - DNA, 20 bp, Zea mays
gcatcaccatcctccttgct

SEQ ID NO: 162 - DNA, 30 bp, Zea mays
gctaatacttgaatacagaaggatggtgat

SEQ ID NO: 163 - DNA, 25 bp, Zea mays
gccaacatattgtcatccgaggata

SEQ ID NO: 164 - DNA, 20 bp, Zea mays
acgcatcaactgcagagaca

SEQ ID NO: 165 - DNA, 23 bp, Zea mays
gaaaagggaccattcaggtatgc

SEQ ID NO: 166 - DNA, 25 bp, Zea mays
tctgcattggaagttcgcttataca

SEQ ID NO: 167 - DNA, 25 bp, Zea mays
gctcgacagcatccaaaataatctg

SEQ ID NO: 168 - DNA, 25 bp, Zea mays
gcgaattgcactggagatttgattg

SEQ ID NO: 169 - DNA, 20 bp, Zea mays
ctgaagatcgggctgcaatg

SEQ ID NO: 170 - DNA, 20 bp, Zea mays
tgctggtacgaagacaagac

SEQ ID NO: 171 - DNA, 24 bp, Zea mays
aaaacaaaagaacaaaagaactac

SEQ ID NO: 172 - DNA, 21 bp, Zea mays
aagcgaaccgggatcaaagat

SEQ ID NO: 173 - DNA, 25 bp, Zea mays
cctacacgtgacttatccccaaaag

SEQ ID NO: 174 - DNA, 19 bp, Zea mays
gctggacaagatcaaggag

SEQ ID NO: 175 - DNA, 20 bp, Zea mays
gctgaattacaatacgcaac

SEQ ID NO: 176 - DNA, 19 bp, Zea mays
cctgcaggctcacgagtag

SEQ ID NO: 177 - DNA, 18 bp, Zea mays
gtgtctgaggcggaaggt

SEQ ID NO: 178 - DNA, 15 bp, Zea mays
ccgccaccggaacct

SEQ ID NO: 179 - DNA, 16 bp, Zea mays
agcagctcgcccttcc

SEQ ID NO: 180 - DNA, 15 bp, Zea mays
cccaccgcacgacca

SEQ ID NO: 181 - DNA, 21 bp, Zea mays
agtctgagccatcaccttcct

SEQ ID NO: 182 - DNA, 24 bp, Zea mays
ggtcgttcttcacattggttagca

SEQ ID NO: 183 - DNA, 17 bp, Zea mays
caccgccgctacagtct

SEQ ID NO: 184 - DNA, 25 bp, Zea mays
cagaaaacgcaacaaactacaacca

SEQ ID NO: 185 - DNA, 25 bp, Zea mays
agtaagcattgctcgtttaggatgt

SEQ ID NO: 186 - DNA, 19 bp, Zea mays
acacgatcgagcacacaag

SEQ ID NO: 187 - DNA, 22 bp, Zea mays
cgtagcataaacagtacacgga

SEQ ID NO: 188 - DNA, 19 bp, Zea mays
gctccaaggcgcatttctg

SEQ ID NO: 189 - DNA, 25 bp, Zea mays
cactctacaggcatctctacatctg

SEQ ID NO: 190 - DNA, 20 bp, Zea mays
caggtcacacaggacaacca

SEQ ID NO: 191 - DNA, 22 bp, Zea mays
ccgagaaatgcgacgtctatgg

SEQ ID NO: 192 - DNA, 22 bp, Zea mays
ccatcgtaggaaccctgtcatc

SEQ ID NO: 193 - DNA, 23 bp, Zea mays
gatgcatgatcagaagggctctt

SEQ ID NO: 194 - DNA, 19 bp, Zea mays
aggccgtcaccaagttcac

SEQ ID NO: 195 - DNA, 18 bp, Zea mays
gccatgagaagcggcaca

SEQ ID NO: 196 - DNA, 24 bp, Zea mays
acccaagtgtttcagtctttcaga

SEQ ID NO: 197 - DNA, 15 bp, Zea mays
cccaccggcgaagga

SEQ ID NO: 198 - DNA, 21 bp, Zea mays
atctgcctctccctgatcaat

SEQ ID NO: 199 - DNA, 21 bp, Zea mays
ctgtagaagccgtgaaggaga

SEQ ID NO: 200 - DNA, 25 bp, Zea mays
tgtaaggtgaagcttttgtcctgat

SEQ ID NO: 201 - DNA, 22 bp, Zea mays
tgactccatgatggcatttcgt

SEQ ID NO: 202 - DNA, 16 bp, Zea mays
acggagtggcgcagag

SEQ ID NO: 203 - DNA, 22 bp, Zea mays
tgctccagctttgacactatcg

SEQ ID NO: 204 - DNA, 25 bp, Zea mays
tctgcacagcatcttaattgtcact

SEQ ID NO: 205 - DNA, 27 bp, Zea mays
gttcaaagggagactaaaaccttaggt

SEQ ID NO: 206 - DNA, 23 bp, Zea mays
ccagggaattgcactcagcttag

SEQ ID NO: 207 - DNA, 23 bp, Zea mays
ctctggcacgtggatttcctaaa

SEQ ID NO: 208 - DNA, 20 bp, Zea mays
cccagctcccacatgaatgt

SEQ ID NO: 209 - DNA, 25 bp, Zea mays
ggaccatgtttcggtctcttcttaa

SEQ ID NO: 210 - DNA, 20 bp, Zea mays
cgtgggatttcccatctctc

SEQ ID NO: 211 - DNA, 20 bp, Zea mays
ccacatttgttgcatccttg

SEQ ID NO: 212 - DNA, 20 bp, Zea mays
gccatcagcacgaacaggat

SEQ ID NO: 213 - DNA, 20 bp, Zea mays
tcgctaccaccaccacctaa

SEQ ID NO: 214 - DNA, 17 bp, Zea mays
ccgagtccgcacaggtt

SEQ ID NO: 215 - DNA, 21 bp, Zea mays
ccgacaggttaggcgtaatcg

SEQ ID NO: 216 - DNA, 22 bp, Zea mays
agcaaaagttcagttctctagc

SEQ ID NO: 217 - DNA, 19 bp, Zea mays
acgacgaagctggagatac

SEQ ID NO: 218 - DNA, 16 bp, Zea mays
ggcacgcgagcatctg

SEQ ID NO: 219 - DNA, 19 bp, Zea mays
ccaccttcgtgtccatcgt

SEQ ID NO: 220 - DNA, 14 bp, Zea mays
gcccggcgctgtca

SEQ ID NO: 221 - DNA, 19 bp, Zea mays
ccatcgcttgccctgtctt

SEQ ID NO: 222 - DNA, 23 bp, Zea mays
tctaggttcattggcacgtactg

SEQ ID NO: 223 - DNA, 19 bp, Zea mays
cccagtctctgcgatgaca

SEQ ID NO: 224 - DNA, 26 bp, Zea mays
ctgttgttatctgtgaggttgatcct

SEQ ID NO: 225 - DNA, 22 bp, Zea mays
acacgtggaaccagttcgttta

SEQ ID NO: 226 - DNA, 28 bp, Zea mays
gatatggatacgtaggcattcctgaatt

SEQ ID NO: 227 - DNA, 33 bp, Zea mays
tgctactgatttcattcagattagatgtttctt

SEQ ID NO: 228 - DNA, 20 bp, Zea mays
tggccatgttgcatgagtga

SEQ ID NO: 229 - DNA, 21 bp, Zea mays
tcagacctgcaagtgctttct

SEQ ID NO: 230 - DNA, 20 bp, Zea mays
ccgaggccgagagcaatatg

SEQ ID NO: 231 - DNA, 19 bp, Zea mays
gcagtcgcatcctggtact

SEQ ID NO: 232 - DNA, 15 bp, Zea mays
ctggaatggcagatc

SEQ ID NO: 233 - DNA, 16 bp, Zea mays
ctggaatgacagatct

SEQ ID NO: 234 - DNA, 15 bp, Zea mays
acagctttgaaggca

SEQ ID NO: 235 - DNA, 14 bp, Zea mays
acagctgtgaaggc

SEQ ID NO: 236 - DNA, 13 bp, Zea mays
cgctctcggtctc

SEQ ID NO: 237 - DNA, 13 bp, Zea mays
cgctctcagtctc

SEQ ID NO: 238 - DNA, 14 bp, Zea mays
atgcatgcgcgcag

SEQ ID NO: 239 - DNA, 16 bp, Zea mays
catatgcatgcagcgc

SEQ ID NO: 240 - DNA, 14 bp, Zea mays
acgagcaacaacca

SEQ ID NO: 241 - DNA, 14 bp, Zea mays
acgagcaacagcca

SEQ ID NO: 242 - DNA, 23 bp, Zea mays
caaagaacaaacttagtactaca

SEQ ID NO: 243 - DNA, 17 bp, Zea mays
acaaacttggaactaca

SEQ ID NO: 244 - DNA, 20 bp, Zea mays
tctttcaggtattccacaaa

SEQ ID NO: 245 - DNA, 20 bp, Zea mays
atctttcaggtcttccacaa

SEQ ID NO: 246 - DNA, 16 bp, Zea mays
atttgagcaccttgtg

SEQ ID NO: 247 - DNA, 16 bp, Zea mays
agatttgcaccttgtg

SEQ ID NO: 248 - DNA, 19 bp, Zea mays
aaaacattcataaagatct

SEQ ID NO: 249 - DNA, 19 bp, Zea mays
aaaacattcatgaagatct

SEQ ID NO: 250 - DNA, 16 bp, Zea mays
aagctcatcaaagaat

SEQ ID NO: 251 - DNA, 16 bp, Zea mays
aagctcatcgaagaat

SEQ ID NO: 252 - DNA, 17 bp, Zea mays
agcttgtcgttccaata

SEQ ID NO: 253 - DNA, 18 bp, Zea mays
agcttgtcattccaataa

SEQ ID NO: 254 - DNA, 17 bp, Zea mays
aaaggctcaatatactg

SEQ ID NO: 255 - DNA, 18 bp, Zea mays
caaaggctcactatactg

SEQ ID NO: 256 - DNA, 21 bp, Zea mays
catgattattgacactagtgt

SEQ ID NO: 257 - DNA, 21 bp, Zea mays
catgattattgacactaatgt

SEQ ID NO: 258 - DNA, 14 bp, Zea mays
caacggctgcactc

SEQ ID NO: 259 - DNA, 17 bp, Zea mays
cttcaacgtctgcactc

SEQ ID NO: 260 - DNA, 14 bp, Zea mays
ctcggccccacctt

SEQ ID NO: 261 - DNA, 13 bp, Zea mays
tcggcccgacctt

SEQ ID NO: 262 - DNA, 16 bp, Zea mays
aacgagcctactctga

SEQ ID NO: 263 - DNA, 16 bp, Zea mays
aacgagccaactctga

SEQ ID NO: 264 - DNA, 17 bp, Zea mays
atgaacgggaaccacga

SEQ ID NO: 265 - DNA, 17 bp, Zea mays
atgaacgggaaccaaga

SEQ ID NO: 266 - DNA, 13 bp, Zea mays
ccatgcagctgtc

SEQ ID NO: 267 - DNA, 13 bp, Zea mays
ccatgcagctctc

SEQ ID NO: 268 - DNA, 19 bp, Zea mays
caagaaaatcgtgttgaag

SEQ ID NO: 269 - DNA, 20 bp, Zea mays
ccaagaaaatcgtattgaag

SEQ ID NO: 270 - DNA, 13 bp, Zea mays
cgatggccgcggc

SEQ ID NO: 271 - DNA, 16 bp, Zea mays
atgcgatagccgcggc

SEQ ID NO: 272 - DNA, 17 bp, Zea mays
actccatcaggcagtgg

SEQ ID NO: 273 - DNA, 17 bp, Zea mays
actccatcaagcagtgg

SEQ ID NO: 274 - DNA, 14 bp, Zea mays
catgcgcgtgtcct

SEQ ID NO: 275 - DNA, 17 bp, Zea mays
aatcatgcgcctgtcct

SEQ ID NO: 276 - DNA, 16 bp, Zea mays
ctggagaaggaaagta

SEQ ID NO: 277 - DNA, 17 bp, Zea mays
cctggagaatgaaagta

SEQ ID NO: 278 - DNA, 17 bp, Zea mays
cagaaagtgccttattt

SEQ ID NO: 279 - DNA, 17 bp, Zea mays
cagaaagtggcttattt

SEQ ID NO: 280 - DNA, 17 bp, Zea mays
atgatctctgagcccgg

SEQ ID NO: 281 - DNA, 17 bp, Zea mays
atgatctctgggcccgg

SEQ ID NO: 282 - DNA, 21 bp, Zea mays
cttttgatttcctttatttgt

SEQ ID NO: 283 - DNA, 21 bp, Zea mays
cttttgatttccttcatttgt

SEQ ID NO: 284 - DNA, 18 bp, Zea mays
ttgtaacatctggttcct

SEQ ID NO: 285 - DNA, 16 bp, Zea mays
tgtaacatgtgcttcc

SEQ ID NO: 286 - DNA, 19 bp, Zea mays
ctgatgagtatcgtgttac

SEQ ID NO: 287 - DNA, 15 bp, Zea mays
tggcgtacgtgttac

SEQ ID NO: 288 - DNA, 14 bp, Zea mays
aacgacagattcgg

SEQ ID NO: 289 - DNA, 14 bp, Zea mays
aacgacggattcgg

SEQ ID NO: 290 - DNA, 16 bp, Zea mays
ctgttgccattccatt

SEQ ID NO: 291 - DNA, 16 bp, Zea mays
ctgttgccgttccatt

SEQ ID NO: 292 - DNA, 15 bp, Zea mays
aatgcaagcattaat

SEQ ID NO: 293 - DNA, 16 bp, Zea mays
caatgcaaacattaat

SEQ ID NO: 294 - DNA, 15 bp, Zea mays
cctccagactgatcc

SEQ ID NO: 295 - DNA, 14 bp, Zea mays
ctccaggctgatcc

SEQ ID NO: 296 - DNA, 15 bp, Zea mays
cggcgagattgtcaa

SEQ ID NO: 297 - DNA, 17 bp, Zea mays
aacggcgaaattgtcaa

SEQ ID NO: 298 - DNA, 16 bp, Zea mays
tagcagcaggtcatgt

SEQ ID NO: 299 - DNA, 17 bp, Zea mays
ctagcagcagatcatgt

SEQ ID NO: 300 - DNA, 15 bp, Zea mays
tccaaggcgctgtat

SEQ ID NO: 301 - DNA, 17 bp, Zea mays
tctccaaggcactgtat

SEQ ID NO: 302 - DNA, 14 bp, Zea mays
ccggcaatagccca

SEQ ID NO: 303 - DNA, 14 bp, Zea mays
ccggcagtagccca

SEQ ID NO: 304 - DNA, 16 bp, Zea mays
ctactccacagttagc

SEQ ID NO: 305 - DNA, 15 bp, Zea mays
ctccacacagttagc

SEQ ID NO: 306 - DNA, 14 bp, Zea mays
caatgccaggtctc

SEQ ID NO: 307 - DNA, 15 bp, Zea mays
ccaatgcctggtctc

SEQ ID NO: 308 - DNA, 17 bp, Zea mays
caagttgttctaaatat

SEQ ID NO: 309 - DNA, 20 bp, Zea mays
ctccaagttgttctatatat

SEQ ID NO: 310 - DNA, 15 bp, Zea mays
ccaagtgagcctaac

SEQ ID NO: 311 - DNA, 15 bp, Zea mays
ccaagtgaacctaac

SEQ ID NO: 312 - DNA, 18 bp, Zea mays
cttattcatggatttatc

SEQ ID NO: 313 - DNA, 18 bp, Zea mays
cttattcatgggtttatc

SEQ ID NO: 314 - DNA, 14 bp, Zea mays
ccgcactgtaccgc

SEQ ID NO: 315 - DNA, 14 bp, Zea mays
ccgcactataccgc

SEQ ID NO: 316 - DNA, 13 bp, Zea mays
ccgcaaagatgaa

SEQ ID NO: 317 - DNA, 13 bp, Zea mays
ccgcagagatgaa

SEQ ID NO: 318 - DNA, 14 bp, Zea mays
cccgtggagtactt

SEQ ID NO: 319 - DNA, 14 bp, Zea mays
cccgtcgagtactt

SEQ ID NO: 320 - DNA, 13 bp, Zea mays
cagcagaagcacc

SEQ ID NO: 321 - DNA, 14 bp, Zea mays
ccagcagcagcacc

SEQ ID NO: 322 - DNA, 16 bp, Zea mays
aaagtgtgcaagatat

SEQ ID NO: 323 - DNA, 18 bp, Zea mays
acaaagtgtgaaagatat

SEQ ID NO: 324 - DNA, 14 bp, Zea mays
cgcctacaacaagg

SEQ ID NO: 325 - DNA, 17 bp, Zea mays
cgacgcctactacaagg

SEQ ID NO: 326 - DNA, 17 bp, Zea mays
cactcgagtgaggtgta

SEQ ID NO: 327 - DNA, 17 bp, Zea mays
cactcgagtgaggtata

SEQ ID NO: 328 - DNA, 15 bp, Zea mays
ttccccagcgacccg

SEQ ID NO: 329 - DNA, 13 bp, Zea mays
ccccagggacccg

SEQ ID NO: 330 - DNA, 15 bp, Zea mays
cagggagactttatt

SEQ ID NO: 331 - DNA, 17 bp, Zea mays
cagggagactttttatt

SEQ ID NO: 332 - DNA, 19 bp, Zea mays
tcgaaccattaagttactt

SEQ ID NO: 333 - DNA, 18 bp, Zea mays
cgaaccattacgttactt

SEQ ID NO: 334 - DNA, 16 bp, Zea mays
catacctatcgatttc

SEQ ID NO: 335 - DNA, 16 bp, Zea mays
catacctatcaatttc

SEQ ID NO: 336 - DNA, 14 bp, Zea mays
ctgcctaccgctcc

SEQ ID NO: 337 - DNA, 17 bp, Zea mays
attctgccttccgctcc

SEQ ID NO: 338 - DNA, 14 bp, Zea mays
ccactgcccctcct

SEQ ID NO: 339 - DNA, 14 bp, Zea mays
ccactggccctcct

SEQ ID NO: 340 - DNA, 16 bp, Zea mays
cttgccttgtgttctg

SEQ ID NO: 341 - DNA, 16 bp, Zea mays
cttgccttctgttctg

SEQ ID NO: 342 - DNA, 14 bp, Zea mays
actcgccagaggtg

SEQ ID NO: 343 - DNA, 14 bp, Zea mays
actcgccggaggtg

SEQ ID NO: 344 - DNA, 15 bp, Zea mays
acagcttacggcggc

SEQ ID NO: 345 - DNA, 13 bp, Zea mays
agcttgcggcggc

SEQ ID NO: 346 - DNA, 17 bp, Zea mays
cttgtgtcaatgcagga

SEQ ID NO: 347 - DNA, 14 bp, Zea mays
ccaaggtcaatgca

SEQ ID NO: 348 - DNA, 14 bp, Zea mays
tcctccgctttcat

SEQ ID NO: 349 - DNA, 14 bp, Zea mays
ctcctccactttca

SEQ ID NO: 350 - DNA, 23 bp, Zea mays
caaagaacaaacttagtactaca

SEQ ID NO: 351 - DNA, 17 bp, Zea mays
acaaacttggaactaca

SEQ ID NO: 352 - DNA, 20 bp, Zea mays
tctttcaggtattccacaaa

SEQ ID NO: 353 - DNA, 20 bp, Zea mays
atctttcaggtcttccacaa

SEQ ID NO: 354 - DNA, 17 bp, Zea mays
cagaaagtgccttattt

SEQ ID NO: 355 - DNA, 17 bp, Zea mays
cagaaagtggcttattt

SEQ ID NO: 356 - DNA, 21 bp, Zea mays
cttttgatttcctttatttgt

SEQ ID NO: 357 - DNA, 21 bp, Zea mays
cttttgatttccttcatttgt

SEQ ID NO: 358 - DNA, 17 bp, Zea mays
acgatgactgccaccca

SEQ ID NO: 359 - DNA, 18 bp, Zea mays
cacgatgactaccaccca

SEQ ID NO: 360 - DNA, 17 bp, Zea mays
ccaaacacaacgaagag

SEQ ID NO: 361 - DNA, 17 bp, Zea mays
ccaaacacgacgaagag

SEQ ID NO: 362 - DNA, 17 bp, Zea mays
cctttaatggccttttt

SEQ ID NO: 363 - DNA, 18 bp, Zea mays
tcctttaatggacttttt

SEQ ID NO: 364 - DNA, 16 bp, Zea mays
ctgttgccattccatt

SEQ ID NO: 365 - DNA, 16 bp, Zea mays
ctgttgccgttccatt

SEQ ID NO: 366 - DNA, 17 bp, Zea mays
cagtagcacgattcata

SEQ ID NO: 367 - DNA, 17 bp, Zea mays
cagtagcacgcttcata

SEQ ID NO: 368 - DNA, 15 bp, Zea mays
aatgcaagcattaat

SEQ ID NO: 369 - DNA, 16 bp, Zea mays
caatgcaaacattaat

SEQ ID NO: 370 - DNA, 20 bp, Zea mays
ttcatacctacattaaagat

SEQ ID NO: 371 - DNA, 18 bp, Zea mays
catacctacatcaaagat

SEQ ID NO: 372 - DNA, 16 bp, Zea mays
atgcagcatatacttt

SEQ ID NO: 373 - DNA, 17 bp, Zea mays
catgcaacatatacttt

SEQ ID NO: 374 - DNA, 15 bp, Zea mays
cagacgcacgtgaac

SEQ ID NO: 375 - DNA, 15 bp, Zea mays
cagacgcccgtgaac

SEQ ID NO: 376 - DNA, 13 bp, Zea mays
ccgacgccggttt

SEQ ID NO: 377 - DNA, 13 bp, Zea mays
ccgacgccggctt

SEQ ID NO: 378 - DNA, 16 bp, Zea mays
attgcaaccgtcaagg

SEQ ID NO: 379 - DNA, 18 bp, Zea mays
tcattgcaaccctcaagg

SEQ ID NO: 380 - DNA, 16 bp, Zea mays
cttgagagtaatcttg

SEQ ID NO: 381 - DNA, 16 bp, Zea mays
cttgagagtgatcttg

SEQ ID NO: 382 - DNA, 15 bp, Zea mays
aagcaacagaaacaa

SEQ ID NO: 383 - DNA, 16 bp, Zea mays
caagcaacaaaaacaa

SEQ ID NO: 384 - DNA, 16 bp, Zea mays
acaccacaggaccata

SEQ ID NO: 385 - DNA, 16 bp, Zea mays
acaccacacgaccata

SEQ ID NO: 386 - DNA, 17 bp, Zea mays
tcgatctcccagtataa

SEQ ID NO: 387 - DNA, 17 bp, Zea mays
tcgatctcccaatataa

SEQ ID NO: 388 - DNA, 16 bp, Zea mays
taggcatccgcagact

SEQ ID NO: 389 - DNA, 16 bp, Zea mays
taggcatcggcagact

SEQ ID NO: 390 - DNA, 15 bp, Zea mays
acgtgctcttcaagc

SEQ ID NO: 391 - DNA, 16 bp, Zea mays
aacgtgctattcaagc

SEQ ID NO: 392 - DNA, 17 bp, Zea mays
tcgacacgatgtgacca

SEQ ID NO: 393 - DNA, 18 bp, Zea mays
ctcgacacgatttgacca

SEQ ID NO: 394 - DNA, 16 bp, Zea mays
atgcatgtacgaactg

SEQ ID NO: 395 - DNA, 17 bp, Zea mays
catgcatgtaagaactg

SEQ ID NO: 396 - DNA, 16 bp, Zea mays
aagcaaccatcagtgc

SEQ ID NO: 397 - DNA, 16 bp, Zea mays
aagcaaccgtcagtgc

SEQ ID NO: 398 - DNA, 19 bp, Zea mays
aatgacctcgtatcggagt

SEQ ID NO: 399 - DNA, 18 bp, Zea mays
atgacctcgtgtcggagt

SEQ ID NO: 400 - DNA, 663 bp, Zea mays
  misc_feature (24)..(641): n is a, c, g, or t
  misc_feature (83)..(83): y is c or t
  misc_feature (119)..(119): m is a or c
  misc_feature (601)..(601): w is a or t
ttcctctataagtacccgccccanatctgcgccattttctcatcgcagaaatcctccgcacttcacagcgtatcatcgttttycatcgctcctactcctancatccagaaaatctgagmggtattgatggcgcccaaggcggagaagaagccggcggcnaagaaggtggcggaggaggagccctcggagaaggcggctccggcggagaaggcccccgcggggaagaagnccaaggcggagaagcggctnccngcgggcaagtcngcnggcaaggagggcggcgacaagaagggnaggaagaaggcgaagaagagcgtggagacctacaagatctacatcttcaaggtcctgaagcaggtgcaccccgacatcggcatctcctccaaggccatgtccatcatgaactccttcatcaacgacatcttcgagaagctcgccncggaggccgccaagctcgcccgntacaacaagaagcccaccatcacctcccgcgagatccagacctccgtccgcctcgtcctccccggcgagctcgccaagcacgccgtctcggagggtaccaaggccgtcaccaagttcacctcgtcntagccnccttgtwgtaggcgtcgttgtnnnctgcttctcaagcaagcactgtnatgtgccgcttctcatggcagt

SEQ ID NO: 401 - DNA, 664 bp, Zea mays; identical to SEQ ID NO: 99

SEQ ID NO: 402 - DNA, 22 bp, Zea mays
agaaatcctccgcaacttcaca

SEQ ID NO: 403 - DNA, 19 bp, Zea mays
cttgggcgccatcaatacc

SEQ ID NO: 404 - DNA, 25 bp, Zea mays
caacttcacagcgtatcatcgtttt

SEQ ID NO: 405 - DNA, 16 bp, Zea mays
gccgccggcttcttct

SEQ ID NO: 406 - DNA, 19 bp, Zea mays
aggccgtcaccaagttcac

SEQ ID NO: 407 - DNA, 18 bp, Zea mays
gccatgagaagcggcaca

SEQ ID NO: 408 - DNA, 18 bp, Zea mays
tcatcgtttttcatcgct

SEQ ID NO: 409 - DNA, 18 bp, Zea mays
tcatcgttttccatcgct

SEQ ID NO: 410 - DNA, 18 bp, Zea mays
aaaatctgagaggtattg

SEQ ID NO: 411 - DNA, 17 bp, Zea mays
aaatctgagcggtattg

SEQ ID NO: 412 - DNA, 14 bp, Zea mays
cgcctacaacaagg

SEQ ID NO: 413 - DNA, 17 bp, Zea mays
cgacgcctactacaagg